European Patent Application EP 4 707 393 A1, published March 11, 2026. Title: DOUBLE-STRANDED SIRNA, CONJUGATE THEREOF AND USE THEREOF. Applicant: CMS RESEARCH & DEVELOPMENT PTE. LTD. The sequence listing filed with the application follows.

SEQUENCE LISTING (97 sequences)

SEQ ID NO: 1 - RNA, 16 nt, synthetic construct
  source 1..16: mol_type = other RNA
cccttattgttatacg

SEQ ID NO: 2 - RNA, 16 nt, synthetic construct
  source 1..16: mol_type = other RNA
ccccttattgttatac

SEQ ID NO: 3 - RNA, 16 nt, synthetic construct
  source 1..16: mol_type = other RNA
gccccttattgttata

SEQ ID NO: 4 - RNA, 16 nt, synthetic construct
  source 1..16: mol_type = other RNA
agccccttattgttat

SEQ ID NO: 5 - RNA, 16 nt, synthetic construct
  source 1..16: mol_type = other RNA
cagccccttattgtta

SEQ ID NO: 6 - RNA, 18 nt, synthetic construct
  source 1..18: mol_type = other RNA
gccccttattgttatacg

SEQ ID NO: 7 - RNA, 18 nt, synthetic construct
  source 1..18: mol_type = other RNA
  modified_base 1: mod_base = OTHER; note = n is R
  modified_base 18: mod_base = OTHER; note = n is R
nccccttattgttatacn

SEQ ID NO: 8 - RNA, 18 nt, synthetic construct
  source 1..18: mol_type = other RNA
  modified_base 11: mod_base = OTHER; note = n is R
gccccttattnttatacg

SEQ ID NO: 9 - RNA, 18 nt, synthetic construct
  source 1..18: mol_type = other RNA
  modified_base 1: mod_base = OTHER; note = n is R
  modified_base 11: mod_base = OTHER; note = n is R
nccccttattnttatacg

SEQ ID NO: 10 - RNA, 19 nt, synthetic construct
  source 1..19: mol_type = other RNA
  modified_base 1: mod_base = OTHER; note = n is R
  modified_base 18: mod_base = OTHER; note = n is R
nccccttattgttatacna

SEQ ID NO: 11 - RNA, 19 nt, synthetic construct
  source 1..19: mol_type = other RNA
  modified_base 1: mod_base = OTHER; note = n is R
  modified_base 19: mod_base = OTHER; note = n is R
nccccttattgttatacgn

SEQ ID NO: 12 - RNA, 21 nt, synthetic construct
  source 1..21: mol_type = other RNA
  modified_base 1: mod_base = OTHER; note = n is R
  modified_base 21: mod_base = OTHER; note = n is R
nccccttattgttatacgagn

SEQ ID NO: 13 - RNA, 21 nt, synthetic construct
  source 1..21: mol_type = other RNA
  modified_base 1: mod_base = OTHER; note = n is R
  modified_base 19: mod_base = OTHER; note = n is R
nccccttattgttatacgnga

SEQ ID NO: 14 - RNA, 17 nt, synthetic construct
  source 1..17: mol_type = other RNA
  modified_base 13: mod_base = OTHER; note = n is R
cccttattgttanacga

SEQ ID NO: 15 - RNA, 21 nt, synthetic construct
  source 1..21: mol_type = other RNA
  modified_base 17: mod_base = OTHER; note = n is R
cagccccttattgttanacga

SEQ ID NO: 16 - RNA, 19 nt, synthetic construct
  source 1..19: mol_type = other RNA
tgccaagcttggtcatcta

SEQ ID NO: 17 - RNA, 18 nt, synthetic construct
  source 1..18: mol_type = other RNA
gccaagcttggtcatcta

SEQ ID NO: 18 - RNA, 20 nt, synthetic construct
  source 1..20: mol_type = other RNA
ttgccaagcttggtcatcta

SEQ ID NO: 19 - RNA, 28 nt, synthetic construct
  source 1..28: mol_type = other RNA
  modified_base 11: mod_base = OTHER; note = n is Z
atccctcgtanaacaataaggggctgtt

SEQ ID NO: 20 - RNA, 23 nt, synthetic construct
  source 1..23: mol_type = other RNA
  modified_base 6: mod_base = OTHER; note = n is Z
tcgtanaacaataaggggctgtt

SEQ ID NO: 21 - RNA, 28 nt, synthetic construct
  source 1..28: mol_type = other RNA
  modified_base 11: mod_base = OTHER; note = n is Z
atccctcgtanaacaataaggggctgcc

SEQ ID NO: 22 - RNA, 25 nt, synthetic construct
  source 1..25: mol_type = other RNA
  modified_base 8: mod_base = OTHER; note = n is Z
tctcgtanaacaataaggggctgtt

SEQ ID NO: 23 - RNA, 23 nt, synthetic construct
  source 1..23: mol_type = other RNA
  modified_base 9: mod_base = OTHER; note = n is R
tctcgtatnacaataaggggctt

SEQ ID NO: 24 - RNA, 23 nt, synthetic construct
  source 1..23: mol_type = other RNA
  modified_base 9: mod_base = OTHER; note = n is R
tctcgtatnacaataaggggctg

SEQ ID NO: 25 - RNA, 21 nt, synthetic construct
  source 1..21: mol_type = other RNA
  modified_base 6: mod_base = OTHER; note = n is R
  modified_base 20: mod_base = OTHER; note = n is R
tagatnaccaagcttggcang

SEQ ID NO: 26 - RNA, 22 nt, synthetic construct
  source 1..22: mol_type = other RNA
  modified_base 6: mod_base = OTHER; note = n is R
  modified_base 20: mod_base = OTHER; note = n is R
tagatnaccaagcttggcangg

SEQ ID NO: 27 - RNA, 16 nt, synthetic construct
  source 1..16: mol_type = other RNA
  modified_base 1..2: mod_base = OTHER; note = 2'-O-methylcytidine
  modified_base 3: mod_base = OTHER; note = 2'-O-methylcytidine
  modified_base 4: mod_base = OTHER; note = 2'-O-methyluridine
  modified_base 5: mod_base = OTHER; note = 2'-fluorouridine
  modified_base 6: mod_base = OTHER; note = 2'-fluoroadenosine
  modified_base 7: mod_base = OTHER; note = 2'-fluorouridine
  modified_base 8: mod_base = OTHER; note = 2'-O-methyluridine
  modified_base 9: mod_base = OTHER; note = 2'-O-methylguanosine
  modified_base 10..11: mod_base = OTHER; note = 2'-O-methyluridine
  modified_base 12: mod_base = OTHER; note = 2'-O-methyladenosine
  modified_base 13: mod_base = OTHER; note = 2'-O-methyluridine
  modified_base 14: mod_base = OTHER; note = 2'-O-methyladenosine
  modified_base 15: mod_base = OTHER; note = 2'-O-methylcytidine
  modified_base 16: mod_base = OTHER; note = 2'-O-methylguanosine
  modified_base 1..2: mod_base = OTHER; note = phosphorothioate linkage
  modified_base 2..3: mod_base = OTHER; note = phosphorothioate linkage
cccttattgttatacg

SEQ ID NO: 28 - RNA, 16 nt, synthetic construct
  source 1..16: mol_type = other RNA
  modified_base 1..2: mod_base = OTHER; note = 2'-O-methylcytidine
  modified_base 3..4: mod_base = OTHER; note = 2'-O-methylcytidine
  modified_base 5: mod_base = OTHER; note = 2'-O-methyluridine
  modified_base 6: mod_base = OTHER; note = 2'-fluorouridine
  modified_base 7: mod_base = OTHER; note = 2'-fluoroadenosine
  modified_base 8: mod_base = OTHER; note = 2'-fluorouridine
  modified_base 9: mod_base = OTHER; note = 2'-O-methyluridine
  modified_base 10: mod_base = OTHER; note = 2'-O-methylguanosine
  modified_base 11..12: mod_base = OTHER; note = 2'-O-methyluridine
  modified_base 13: mod_base = OTHER; note = 2'-O-methyladenosine
  modified_base 14: mod_base = OTHER; note = 2'-O-methyluridine
  modified_base 15: mod_base = OTHER; note = 2'-O-methyladenosine
  modified_base 16: mod_base = OTHER; note = 2'-O-methylcytidine
  modified_base 1..2: mod_base = OTHER; note = phosphorothioate linkage
  modified_base 2..3: mod_base = OTHER; note = phosphorothioate linkage
ccccttattgttatac

SEQ ID NO: 29 - RNA, 16 nt, synthetic construct
  source 1..16: mol_type = other RNA
  modified_base 1: mod_base = OTHER; note = 2'-O-methylguanosine
  modified_base 2: mod_base = OTHER; note = 2'-O-methylcytidine
  modified_base 3..5: mod_base = OTHER; note = 2'-O-methylcytidine
  modified_base 6: mod_base = OTHER; note = 2'-O-methyluridine
  modified_base 7: mod_base = OTHER; note = 2'-fluorouridine
  modified_base 8: mod_base = OTHER; note = 2'-fluoroadenosine
  modified_base 9: mod_base = OTHER; note = 2'-fluorouridine
  modified_base 10: mod_base = OTHER; note = 2'-O-methyluridine
  modified_base 11: mod_base = OTHER; note = 2'-O-methylguanosine
  modified_base 12..13: mod_base = OTHER; note = 2'-O-methyluridine
  modified_base 14: mod_base = OTHER; note = 2'-O-methyladenosine
  modified_base 15: mod_base = OTHER; note = 2'-O-methyluridine
  modified_base 16: mod_base = OTHER; note = 2'-O-methyladenosine
  modified_base 1..2: mod_base = OTHER; note = phosphorothioate linkage
  modified_base 2..3: mod_base = OTHER; note = phosphorothioate linkage
gccccttattgttata

SEQ ID NO: 30 - RNA, 16 nt, synthetic construct
  source 1..16: mol_type = other RNA
  modified_base 1: mod_base = OTHER; note = 2'-O-methyladenosine
  modified_base 2: mod_base = OTHER; note = 2'-O-methylguanosine
  modified_base 3..6: mod_base = OTHER; note = 2'-O-methylcytidine
  modified_base 7: mod_base = OTHER; note = 2'-O-methyluridine
  modified_base 8: mod_base = OTHER; note = 2'-fluorouridine
  modified_base 9: mod_base = OTHER; note = 2'-fluoroadenosine
  modified_base 10: mod_base = OTHER; note = 2'-fluorouridine
  modified_base 11: mod_base = OTHER; note = 2'-O-methyluridine
  modified_base 12: mod_base = OTHER; note = 2'-O-methylguanosine
  modified_base 13..14: mod_base = OTHER; note = 2'-O-methyluridine
  modified_base 15: mod_base = OTHER; note = 2'-O-methyladenosine
  modified_base 16: mod_base = OTHER; note = 2'-O-methyluridine
  modified_base 1..2: mod_base = OTHER; note = phosphorothioate linkage
  modified_base 2..3: mod_base = OTHER; note = phosphorothioate linkage
agccccttattgttat

SEQ ID NO: 31 - RNA, 16 nt, synthetic construct
  source 1..16: mol_type = other RNA
  modified_base 1: mod_base = OTHER; note = 2'-O-methylcytidine
  modified_base 2: mod_base = OTHER; note = 2'-O-methyladenosine
  modified_base 3: mod_base = OTHER; note = 2'-O-methylguanosine
  modified_base 4..7: mod_base = OTHER; note = 2'-O-methylcytidine
  modified_base 8: mod_base = OTHER; note = 2'-O-methyluridine
  modified_base 9: mod_base = OTHER; note = 2'-fluorouridine
  modified_base 10: mod_base = OTHER; note = 2'-fluoroadenosine
  modified_base 11: mod_base = OTHER; note = 2'-fluorouridine
  modified_base 12: mod_base = OTHER; note = 2'-O-methyluridine
  modified_base 13: mod_base = OTHER; note = 2'-O-methylguanosine
  modified_base 14..15: mod_base = OTHER; note = 2'-O-methyluridine
  modified_base 16: mod_base = OTHER; note = 2'-O-methyladenosine
  modified_base 1..2: mod_base = OTHER; note = phosphorothioate linkage
  modified_base 2..3: mod_base = OTHER; note = phosphorothioate linkage
cagccccttattgtta

SEQ ID NO: 32 - RNA, 16 nt, synthetic construct
  source 1..16: mol_type = other RNA
  modified_base 1..2: mod_base = OTHER; note = 2'-O-methylcytidine
  modified_base 3: mod_base = OTHER; note = 2'-O-methylcytidine
  modified_base 4..5: mod_base = OTHER; note = 2'-O-methyluridine
  modified_base 6: mod_base = OTHER; note = 2'-fluoroadenosine
  modified_base 7..8: mod_base = OTHER; note = 2'-fluorouridine
  modified_base 9: mod_base = OTHER; note = 2'-O-methylguanosine
  modified_base 10..11: mod_base = OTHER; note = 2'-O-methyluridine
  modified_base 12: mod_base = OTHER; note = 2'-O-methyladenosine
  modified_base 13: mod_base = OTHER; note = 2'-O-methyluridine
  modified_base 14: mod_base = OTHER; note = 2'-O-methyladenosine
  modified_base 15: mod_base = OTHER; note = 2'-O-methylcytidine
  modified_base 16: mod_base = OTHER; note = 2'-O-methylguanosine
  modified_base 1..2: mod_base = OTHER; note = phosphorothioate linkage
  modified_base 2..3: mod_base = OTHER; note = phosphorothioate linkage
cccttattgttatacg

SEQ ID NO: 33 - RNA, 16 nt, synthetic construct
  source 1..16: mol_type = other RNA
  modified_base 1..2: mod_base = OTHER; note = 2'-O-methylcytidine
  modified_base 3: mod_base = OTHER; note = 2'-O-methylcytidine
  modified_base 4..5: mod_base = OTHER; note = 2'-O-methyluridine
  modified_base 6: mod_base = OTHER; note = 2'-O-methyladenosine
  modified_base 7..8: mod_base = OTHER; note = 2'-fluorouridine
  modified_base 9: mod_base = OTHER; note = 2'-fluoroguanosine
  modified_base 10..11: mod_base = OTHER; note = 2'-O-methyluridine
  modified_base 12: mod_base = OTHER; note = 2'-O-methyladenosine
  modified_base 13: mod_base = OTHER; note = 2'-O-methyluridine
  modified_base 14: mod_base = OTHER; note = 2'-O-methyladenosine
  modified_base 15: mod_base = OTHER; note = 2'-O-methylcytidine
  modified_base 16: mod_base = OTHER; note = 2'-O-methylguanosine
  modified_base 1..2: mod_base = OTHER; note = phosphorothioate linkage
  modified_base 2..3: mod_base = OTHER; note = phosphorothioate linkage
cccttattgttatacg

SEQ ID NO: 34 - RNA, 16 nt, synthetic construct
  source 1..16: mol_type = other RNA
  modified_base 1..2: mod_base = OTHER; note = 2'-O-methylcytidine
  modified_base 3: mod_base = OTHER; note = 2'-O-methylcytidine
  modified_base 4..5: mod_base = OTHER; note = 2'-O-methyluridine
  modified_base 6: mod_base = OTHER; note = 2'-O-methyladenosine
  modified_base 7: mod_base = OTHER; note = 2'-O-methyluridine
  modified_base 8: mod_base = OTHER; note = 2'-fluorouridine
  modified_base 9: mod_base = OTHER; note = 2'-fluoroguanosine
  modified_base 10: mod_base = OTHER; note = 2'-fluorouridine
  modified_base 11: mod_base = OTHER; note = 2'-O-methyluridine
  modified_base 12: mod_base = OTHER; note = 2'-O-methyladenosine
  modified_base 13: mod_base = OTHER; note = 2'-O-methyluridine
  modified_base 14: mod_base = OTHER; note = 2'-O-methyladenosine
  modified_base 15: mod_base = OTHER; note = 2'-O-methylcytidine
  modified_base 16: mod_base = OTHER; note = 2'-O-methylguanosine
  modified_base 1..2: mod_base = OTHER; note = phosphorothioate linkage
  modified_base 2..3: mod_base = OTHER; note = phosphorothioate linkage
cccttattgttatacg

SEQ ID NO: 35 - RNA, 17 nt, synthetic construct
  source 1..17: mol_type = other RNA
  modified_base 1: mod_base = OTHER; note = n is invAb
  modified_base 2: mod_base = OTHER; note = 2'-O-methylcytidine
  modified_base 3..4: mod_base = OTHER; note = 2'-O-methylcytidine
  modified_base 5: mod_base = OTHER; note = 2'-O-methyluridine
  modified_base 6: mod_base = OTHER; note = 2'-fluorouridine
  modified_base 7: mod_base = OTHER; note = 2'-fluoroadenosine
  modified_base 8: mod_base = OTHER; note = 2'-fluorouridine
  modified_base 9: mod_base = OTHER; note = 2'-O-methyluridine
  modified_base 10: mod_base = OTHER; note = 2'-O-methylguanosine
  modified_base 11..12: mod_base = OTHER; note = 2'-O-methyluridine
  modified_base 13: mod_base = OTHER; note = 2'-O-methyladenosine
  modified_base 14: mod_base = OTHER; note = 2'-O-methyluridine
  modified_base 15: mod_base = OTHER; note = 2'-O-methyladenosine
  modified_base 16: mod_base = OTHER; note = 2'-O-methylcytidine
  modified_base 17: mod_base = OTHER; note = 2'-O-methylguanosine
  modified_base 1..2: mod_base = OTHER; note = phosphorothioate linkage
  modified_base 2..3: mod_base = OTHER; note = phosphorothioate linkage
ncccttattgttatacg

SEQ ID NO: 36 - RNA, 19 nt, synthetic construct
  source 1..19: mol_type = other RNA
  modified_base 1: mod_base = OTHER; note = n is invAb
  modified_base 2: mod_base = OTHER; note = n is R
  modified_base 3..6: mod_base = OTHER; note = 2'-O-methylcytidine
  modified_base 7: mod_base = OTHER; note = 2'-O-methyluridine
  modified_base 8: mod_base = OTHER; note = 2'-fluorouridine
  modified_base 9: mod_base = OTHER; note = 2'-fluoroadenosine
  modified_base 10: mod_base = OTHER; note = 2'-fluorouridine
  modified_base 11: mod_base = OTHER; note = 2'-O-methyluridine
  modified_base 12: mod_base = OTHER; note = 2'-O-methylguanosine
  modified_base 13..14: mod_base = OTHER; note = 2'-O-methyluridine
  modified_base 15: mod_base = OTHER; note = 2'-O-methyladenosine
  modified_base 16: mod_base = OTHER; note = 2'-O-methyluridine
  modified_base 17: mod_base = OTHER; note = 2'-O-methyladenosine
  modified_base 18: mod_base = OTHER; note = 2'-O-methylcytidine
  modified_base 19: mod_base = OTHER; note = n is R
  modified_base 1..2: mod_base = OTHER; note = phosphorothioate linkage
  modified_base 2..3: mod_base = OTHER; note = phosphorothioate linkage
nnccccttattgttatacn

SEQ ID NO: 37 - RNA, 20 nt, synthetic construct
  source 1..20: mol_type = other RNA
  modified_base 1: mod_base = OTHER; note = n is invAb
  modified_base 2: mod_base = OTHER; note = n is R
  modified_base 3: mod_base = OTHER; note = 2'-O-methylguanosine
  modified_base 4..7: mod_base = OTHER; note = 2'-O-methylcytidine
  modified_base 8: mod_base = OTHER; note = 2'-O-methyluridine
  modified_base 9: mod_base = OTHER; note = 2'-fluorouridine
  modified_base 10: mod_base = OTHER; note = 2'-fluoroadenosine
  modified_base 11: mod_base = OTHER; note = 2'-fluorouridine
  modified_base 12: mod_base = OTHER; note = 2'-O-methyluridine
  modified_base 13: mod_base = OTHER; note = 2'-O-methylguanosine
  modified_base 14..15: mod_base = OTHER; note = 2'-O-methyluridine
  modified_base 16: mod_base = OTHER; note = 2'-O-methyladenosine
  modified_base 17: mod_base = OTHER; note = 2'-O-methyluridine
  modified_base 18: mod_base = OTHER; note = 2'-O-methyladenosine
  modified_base 19: mod_base = OTHER; note = 2'-O-methylcytidine
  modified_base 20: mod_base = OTHER; note = n is R
  modified_base 1..2: mod_base = OTHER; note = phosphorothioate linkage
  modified_base 2..3: mod_base = OTHER; note = phosphorothioate linkage
nngccccttattgttatacn

SEQ ID NO: 38 - RNA, 20 nt, synthetic construct
  source 1..20: mol_type = other RNA
  modified_base 1: mod_base = OTHER; note = n is invAb
  modified_base 2: mod_base = OTHER; note = n is R
  modified_base 3..6: mod_base = OTHER; note = 2'-O-methylcytidine
  modified_base 7: mod_base = OTHER; note = 2'-O-methyluridine
  modified_base 8: mod_base = OTHER; note = 2'-fluorouridine
  modified_base 9: mod_base = OTHER; note = 2'-fluoroadenosine
  modified_base 10: mod_base = OTHER; note = 2'-fluorouridine
  modified_base 11: mod_base = OTHER; note = 2'-O-methyluridine
  modified_base 12: mod_base = OTHER; note = 2'-O-methylguanosine
  modified_base 13..14: mod_base = OTHER; note = 2'-O-methyluridine
  modified_base 15: mod_base = OTHER; note = 2'-O-methyladenosine
  modified_base 16: mod_base = OTHER; note = 2'-O-methyluridine
  modified_base 17: mod_base = OTHER; note = 2'-O-methyladenosine
  modified_base 18: mod_base = OTHER; note = 2'-O-methylcytidine
  modified_base 19: mod_base = OTHER; note = n is R
  modified_base 20: mod_base = OTHER; note = 2'-O-methyladenosine
  modified_base 1..2: mod_base = OTHER; note = phosphorothioate linkage
  modified_base 2..3: mod_base = OTHER; note = phosphorothioate linkage
nnccccttattgttatacna

SEQ ID NO: 39 - RNA, 20 nt, synthetic construct
  source 1..20: mol_type = other RNA
  modified_base 1: mod_base = OTHER; note = n is invAb
  modified_base 2: mod_base = OTHER; note = n is R
  modified_base 3..6: mod_base = OTHER; note = 2'-O-methylcytidine
  modified_base 7: mod_base = OTHER; note = 2'-O-methyluridine
  modified_base 8: mod_base = OTHER; note = 2'-fluorouridine
  modified_base 9: mod_base = OTHER; note = 2'-fluoroadenosine
  modified_base 10: mod_base = OTHER; note = 2'-fluorouridine
  modified_base 11: mod_base = OTHER; note = 2'-O-methyluridine
  modified_base 12: mod_base = OTHER; note = 2'-O-methylguanosine
  modified_base 13..14: mod_base = OTHER; note = 2'-O-methyluridine
  modified_base 15: mod_base = OTHER; note = 2'-O-methyladenosine
  modified_base 16: mod_base = OTHER; note = 2'-O-methyluridine
  modified_base 17: mod_base = OTHER; note = 2'-O-methyladenosine
  modified_base 18: mod_base = OTHER; note = 2'-O-methylcytidine
  modified_base 19: mod_base = OTHER; note = 2'-O-methylguanosine
  modified_base 20: mod_base = OTHER; note = n is R
  modified_base 1..2: mod_base = OTHER; note = phosphorothioate linkage
  modified_base 2..3: mod_base = OTHER; note = phosphorothioate linkage
nnccccttattgttatacgn

SEQ ID NO: 40 - RNA, 22 nt, synthetic construct
  source 1..22: mol_type = other RNA
  modified_base 1: mod_base = OTHER; note = n is invAb
  modified_base 2: mod_base = OTHER; note = n is R
  modified_base 3..6: mod_base = OTHER; note = 2'-O-methylcytidine
  modified_base 7: mod_base = OTHER; note = 2'-O-methyluridine
  modified_base 8: mod_base = OTHER; note = 2'-fluorouridine
  modified_base 9: mod_base = OTHER; note = 2'-fluoroadenosine
  modified_base 10: mod_base = OTHER; note = 2'-fluorouridine
  modified_base 11: mod_base = OTHER; note = 2'-O-methyluridine
  modified_base 12: mod_base = OTHER; note = 2'-O-methylguanosine
  modified_base 13..14: mod_base = OTHER; note = 2'-O-methyluridine
  modified_base 15: mod_base = OTHER; note = 2'-O-methyladenosine
  modified_base 16: mod_base = OTHER; note = 2'-O-methyluridine
  modified_base 17: mod_base = OTHER; note = 2'-O-methyladenosine
  modified_base 18: mod_base = OTHER; note = 2'-O-methylcytidine
  modified_base 19: mod_base = OTHER; note = 2'-O-methylguanosine
  modified_base 20: mod_base = OTHER; note = 2'-O-methyladenosine
  modified_base 21: mod_base = OTHER; note = 2'-O-methylguanosine
  modified_base 22: mod_base = OTHER; note = n is R
  modified_base 1..2: mod_base = OTHER; note = phosphorothioate linkage
  modified_base 2..3: mod_base = OTHER; note = phosphorothioate linkage
nnccccttattgttatacgagn

SEQ ID NO: 41 - RNA, 22 nt, synthetic construct
  source 1..22: mol_type = other RNA
  modified_base 1: mod_base = OTHER; note = n is invAb
  modified_base 2: mod_base = OTHER; note = n is R
  modified_base 3..6: mod_base = OTHER; note = 2'-O-methylcytidine
  modified_base 7: mod_base = OTHER; note = 2'-O-methyluridine
  modified_base 8: mod_base = OTHER; note = 2'-fluorouridine
  modified_base 9: mod_base = OTHER; note = 2'-fluoroadenosine
  modified_base 10: mod_base = OTHER; note = 2'-fluorouridine
  modified_base 11: mod_base = OTHER; note = 2'-O-methyluridine
  modified_base 12: mod_base = OTHER; note = 2'-O-methylguanosine
  modified_base 13..14: mod_base = OTHER; note = 2'-O-methyluridine
  modified_base 15: mod_base = OTHER; note = 2'-O-methyladenosine
  modified_base 16: mod_base = OTHER; note = 2'-O-methyluridine
  modified_base 17: mod_base = OTHER; note = 2'-O-methyladenosine
  modified_base 18: mod_base = OTHER; note = 2'-O-methylcytidine
  modified_base 19: mod_base = OTHER; note = 2'-O-methylguanosine
  modified_base 20: mod_base = OTHER; note = n is R
  modified_base 21: mod_base = OTHER; note = 2'-O-methylguanosine
  modified_base 22: mod_base = OTHER; note = 2'-O-methyladenosine
  modified_base 1..2: mod_base = OTHER; note = phosphorothioate linkage
  modified_base 2..3: mod_base = OTHER; note = phosphorothioate linkage
nnccccttattgttatacgnga

SEQ ID NO: 42 - RNA, 17 nt, synthetic construct
  source 1..17: mol_type = other RNA
  modified_base 1..2: mod_base = OTHER; note = 2'-O-methylcytidine
  modified_base 3: mod_base = OTHER; note = 2'-O-methylcytidine
  modified_base 4: mod_base = OTHER; note = 2'-O-methyluridine
  modified_base 5: mod_base = OTHER; note = 2'-fluorouridine
  modified_base 6: mod_base = OTHER; note = 2'-fluoroadenosine
  modified_base 7: mod_base = OTHER; note = 2'-fluorouridine
  modified_base 8: mod_base = OTHER; note = 2'-O-methyluridine
  modified_base 9: mod_base = OTHER; note = 2'-O-methylguanosine
  modified_base 10..11: mod_base = OTHER; note = 2'-O-methyluridine
  modified_base 12: mod_base = OTHER; note = 2'-O-methyladenosine
  modified_base 13: mod_base = OTHER; note = n is R
  modified_base 14: mod_base = OTHER; note = 2'-O-methyladenosine
  modified_base 15: mod_base = OTHER; note = 2'-O-methylcytidine
  modified_base 16: mod_base = OTHER; note = 2'-O-methylguanosine
  modified_base 17: mod_base = OTHER; note = 2'-O-methyladenosine
  modified_base 1..2: mod_base = OTHER; note = phosphorothioate linkage
  modified_base 2..3: mod_base = OTHER; note = phosphorothioate linkage
cccttattgttanacga

SEQ ID NO: 43 - RNA, 21 nt, synthetic construct
  source 1..21: mol_type = other RNA
  modified_base 1: mod_base = OTHER; note = 2'-O-methylcytidine
  modified_base 2: mod_base = OTHER; note = 2'-O-methyladenosine
  modified_base 3: mod_base = OTHER; note = 2'-O-methylguanosine
  modified_base 4..7: mod_base = OTHER; note = 2'-O-methylcytidine
  modified_base 8: mod_base = OTHER; note = 2'-O-methyluridine
  modified_base 9: mod_base = OTHER; note = 2'-fluorouridine
  modified_base 10: mod_base = OTHER; note = 2'-fluoroadenosine
  modified_base 11: mod_base = OTHER; note = 2'-fluorouridine
  modified_base 12: mod_base = OTHER; note = 2'-O-methyluridine
  modified_base 13: mod_base = OTHER; note = 2'-O-methylguanosine
  modified_base 14..15: mod_base = OTHER; note = 2'-O-methyluridine
  modified_base 16: mod_base = OTHER; note = 2'-O-methyladenosine
  modified_base 17: mod_base = OTHER; note = n is R
  modified_base 18: mod_base = OTHER; note = 2'-O-methyladenosine
  modified_base 19: mod_base = OTHER; note = 2'-O-methylcytidine
  modified_base 20: mod_base = OTHER; note = 2'-O-methylguanosine
  modified_base 21: mod_base = OTHER; note = 2'-O-methyladenosine
  modified_base 1..2: mod_base = OTHER; note = phosphorothioate linkage
  modified_base 2..3: mod_base = OTHER; note = phosphorothioate linkage
cagccccttattgttanacga

SEQ ID NO: 44 - RNA, 19 nt, synthetic construct
  source 1..19: mol_type = other RNA
  modified_base 1: mod_base = OTHER; note = 2'-O-methyluridine
  modified_base 2: mod_base = OTHER; note = 2'-O-methylguanosine
  modified_base 3..4: mod_base = OTHER; note = 2'-O-methylcytidine
  modified_base 5: mod_base = OTHER; note = 2'-O-methyladenosine
  modified_base 6: mod_base = OTHER; note = 2'-fluoroadenosine
  modified_base 7: mod_base = OTHER; note = 2'-O-methylguanosine
  modified_base 8: mod_base = OTHER; note = 2'-fluorocytidine
  modified_base 9..10: mod_base = OTHER; note = 2'-fluorouridine
  modified_base 11..12: mod_base = OTHER; note = 2'-O-methylguanosine
  modified_base 13: mod_base = OTHER; note = 2'-O-methyluridine
  modified_base 14: mod_base = OTHER; note = 2'-O-methylcytidine
  modified_base 15: mod_base = OTHER; note = 2'-O-methyladenosine
  modified_base 16: mod_base = OTHER; note = 2'-O-methyluridine
  modified_base 17: mod_base = OTHER; note = 2'-O-methylcytidine
  modified_base 18: mod_base = OTHER; note = 2'-O-methyluridine
  modified_base 19: mod_base = OTHER; note = 2'-O-methyladenosine
  modified_base 1..2: mod_base = OTHER; note = phosphorothioate linkage
  modified_base 2..3: mod_base = OTHER; note = phosphorothioate linkage
tgccaagcttggtcatcta

SEQ ID NO: 45 - RNA, 18 nt, synthetic construct
  source 1..18: mol_type = other RNA
  modified_base 1: mod_base = OTHER; note = 2'-O-methylguanosine
  modified_base 2: mod_base = OTHER; note = 2'-O-methylcytidine
  modified_base 3: mod_base = OTHER; note = 2'-O-methylcytidine
  modified_base 4: mod_base = OTHER; note = 2'-fluoroadenosine
  modified_base 5: mod_base = OTHER; note = 2'-O-methyladenosine
  modified_base 6: mod_base = OTHER; note = 2'-fluoroguanosine
  modified_base 7: mod_base = OTHER; note = 2'-fluorocytidine
  modified_base 8: mod_base = OTHER; note = 2'-fluorouridine
  modified_base 9: mod_base = OTHER; note = 2'-O-methyluridine
  modified_base 10..11: mod_base = OTHER; note = 2'-O-methylguanosine
  modified_base 12: mod_base = OTHER; note = 2'-O-methyluridine
  modified_base 13: mod_base = OTHER; note = 2'-O-methylcytidine
  modified_base 14: mod_base = OTHER; note = 2'-O-methyladenosine
  modified_base 15: mod_base = OTHER; note = 2'-O-methyluridine
  modified_base 16: mod_base = OTHER; note = 2'-O-methylcytidine
  modified_base 17: mod_base = OTHER; note = 2'-O-methyluridine
  modified_base 18: mod_base = OTHER; note = 2'-O-methyladenosine
  modified_base 1..2: mod_base = OTHER; note = phosphorothioate linkage
  modified_base 2..3: mod_base = OTHER; note = phosphorothioate linkage
gccaagcttggtcatcta

SEQ ID NO: 46 - RNA, 20 nt, synthetic construct
  source 1..20: mol_type = other RNA
  modified_base 1: mod_base = OTHER; note = 2'-O-methyluridine
  modified_base 2: mod_base = OTHER; note = 2'-O-methyluridine
  modified_base 3: mod_base = OTHER; note = 2'-O-methylguanosine
  modified_base 4..5: mod_base = OTHER; note = 2'-O-methylcytidine
  modified_base 6..7: mod_base = OTHER; note = 2'-O-methyladenosine
  modified_base 8: mod_base = OTHER; note = 2'-fluoroguanosine
  modified_base 9: mod_base = OTHER; note = 2'-fluorocytidine
  modified_base 10..11: mod_base = OTHER; note = 2'-fluorouridine
  modified_base 12..13: mod_base = OTHER; note = 2'-O-methylguanosine
  modified_base 14: mod_base = OTHER; note = 2'-O-methyluridine
  modified_base 15: mod_base = OTHER; note = 2'-O-methylcytidine
  modified_base 16: mod_base = OTHER; note = 2'-O-methyladenosine
  modified_base 17: mod_base = OTHER; note = 2'-O-methyluridine
  modified_base 18: mod_base = OTHER; note = 2'-O-methylcytidine
  modified_base 19: mod_base = OTHER; note = 2'-O-methyluridine
  modified_base 20: mod_base = OTHER; note = 2'-O-methyladenosine
  modified_base 1..2: mod_base = OTHER; note = phosphorothioate linkage
ttgccaagcttggtcatcta

SEQ ID NO: 47 - RNA, 19 nt, synthetic construct
  source 1..19: mol_type = other RNA
  modified_base 1: mod_base = OTHER; note = 2'-O-methylguanosine
  modified_base 2: mod_base = OTHER; note = 2'-O-methylcytidine
  modified_base 3..5: mod_base = OTHER; note = 2'-O-methylcytidine
  modified_base 6: mod_base = OTHER; note = 2'-O-methyluridine
  modified_base 7: mod_base = OTHER; note = 2'-fluorouridine
  modified_base 8: mod_base = OTHER; note = 2'-fluoroadenosine
  modified_base 9: mod_base = OTHER; note = 2'-fluorouridine
  modified_base 10: mod_base = OTHER; note = 2'-O-methyluridine
  modified_base 11: mod_base = OTHER; note = 2'-O-methylguanosine
  modified_base 12..13: mod_base = OTHER; note = 2'-O-methyluridine
  modified_base 14: mod_base = OTHER; note = 2'-O-methyladenosine
  modified_base 15: mod_base = OTHER; note = n is R
  modified_base 16: mod_base = OTHER; note = 2'-O-methyladenosine
  modified_base 17: mod_base = OTHER; note = 2'-O-methylcytidine
  modified_base 18: mod_base = OTHER; note = 2'-O-methylguanosine
  modified_base 19: mod_base = OTHER; note = 2'-O-methyladenosine
  modified_base 1..2: mod_base = OTHER; note = phosphorothioate linkage
  modified_base 2..3: mod_base = OTHER; note = phosphorothioate linkage
gccccttattgttanacga

SEQ ID NO: 48 - RNA, 21 nt, synthetic construct
  source 1..21: mol_type = other RNA
  modified_base 1: mod_base = OTHER; note = 2'-O-methylcytidine
  modified_base 2: mod_base = OTHER; note = 2'-O-methyladenosine
  modified_base 3: mod_base = OTHER; note = 2'-O-methylguanosine
  modified_base 4..6: mod_base = OTHER; note = 2'-O-methylcytidine
  modified_base 7: mod_base = OTHER; note = 2'-fluorocytidine
  modified_base 8: mod_base = OTHER; note = 2'-O-methyluridine
  modified_base 9: mod_base = OTHER; note = 2'-fluorouridine
  modified_base 10: mod_base = OTHER; note = 2'-fluoroadenosine
  modified_base 11: mod_base = OTHER; note = 2'-fluorouridine
  modified_base 12: mod_base = OTHER; note = 2'-O-methyluridine
  modified_base 13: mod_base = OTHER; note = 2'-O-methylguanosine
  modified_base 14..15: mod_base = OTHER; note = 2'-O-methyluridine
  modified_base 16: mod_base = OTHER; note = 2'-O-methyladenosine
  modified_base 17: mod_base = OTHER; note = n is R
  modified_base 18: mod_base = OTHER; note = 2'-O-methyladenosine
  modified_base 19: mod_base = OTHER; note = 2'-O-methylcytidine
  modified_base 20: mod_base = OTHER; note = 2'-O-methylguanosine
  modified_base 21: mod_base = OTHER; note = 2'-O-methyladenosine
  modified_base 1..2: mod_base = OTHER; note = phosphorothioate linkage
  modified_base 2..3: mod_base = OTHER; note = phosphorothioate linkage
cagccccttattgttanacga

SEQ ID NO: 49 - RNA, 21 nt, synthetic construct
  source 1..21: mol_type = other RNA
  modified_base 1: mod_base = OTHER; note = 2'-O-methylcytidine
  modified_base 2: mod_base = OTHER; note = 2'-O-methyladenosine
  modified_base 3: mod_base = OTHER; note = 2'-O-methylguanosine
  modified_base 4..7: mod_base = OTHER; note = 2'-O-methylcytidine
  modified_base 8: mod_base = OTHER; note = 2'-O-methyluridine
  modified_base 9: mod_base = OTHER; note = 2'-fluorouridine
  modified_base 10: mod_base = OTHER; note = 2'-fluoroadenosine
  modified_base 11: mod_base = OTHER; note = 2'-fluorouridine
  modified_base 12: mod_base = OTHER; note = 2'-O-methyluridine
  modified_base 13: mod_base = OTHER; note = 2'-O-methylguanosine
  modified_base 14..15: mod_base = OTHER; note = 2'-O-methyluridine
  modified_base 16: mod_base = OTHER; note = 2'-O-methyladenosine
  modified_base 17: mod_base = OTHER; note = 2'-O-methyluridine
  modified_base 18: mod_base = OTHER; note = 2'-O-methyladenosine
  modified_base 19: mod_base = OTHER; note = 2'-O-methylcytidine
  modified_base 20: mod_base = OTHER; note = 2'-O-methylguanosine
  modified_base 21: mod_base = OTHER; note = 2'-O-methyladenosine
  modified_base 1..2: mod_base = OTHER; note = phosphorothioate linkage
  modified_base 2..3: mod_base = OTHER; note = phosphorothioate linkage
cagccccttattgttatacga

SEQ ID NO: 50 - RNA, 21 nt, synthetic construct
  source 1..21: mol_type = other RNA
  modified_base 1..2: mod_base = OTHER; note = 2'-O-methylcytidine
  modified_base 3: mod_base = OTHER; note = 2'-O-methyluridine
  modified_base 4: mod_base = OTHER; note = 2'-O-methylguanosine
  modified_base 5..6: mod_base = OTHER; note = 2'-O-methylcytidine
  modified_base 7: mod_base = OTHER; note = 2'-fluoroadenosine
  modified_base 8: mod_base = OTHER; note = 2'-O-methyladenosine
  modified_base 9: mod_base = OTHER; note = 2'-fluoroguanosine
  modified_base 10: mod_base = OTHER; note = 2'-fluorocytidine
  modified_base 11: mod_base = OTHER; note = 2'-fluorouridine
  modified_base 12: mod_base = OTHER; note = 2'-O-methyluridine
  modified_base 13..14: mod_base = OTHER; note = 2'-O-methylguanosine
  modified_base 15: mod_base = OTHER; note = 2'-O-methyluridine
  modified_base 16: mod_base = OTHER; note = 2'-O-methylcytidine
  modified_base 17: mod_base = OTHER; note = 2'-O-methyladenosine
  modified_base 18: mod_base = OTHER; note = 2'-O-methyluridine
  modified_base 19: mod_base = OTHER; note = 2'-O-methylcytidine
  modified_base 20: mod_base = OTHER; note = 2'-O-methyluridine
  modified_base 21: mod_base = OTHER; note = 2'-O-methyladenosine
  modified_base 1..2: mod_base = OTHER; note = phosphorothioate linkage
  modified_base 2..3: mod_base = OTHER; note = phosphorothioate linkage
cctgccaagcttggtcatcta

SEQ ID NO: 51 - RNA, 21 nt, synthetic construct
  source 1..21: mol_type = other RNA
  modified_base 1..2: mod_base = OTHER; note = 2'-O-methylcytidine
  modified_base 3: mod_base = OTHER; note = 2'-O-methyluridine
  modified_base 4: mod_base = OTHER; note = 2'-O-methylguanosine
  modified_base 5..6: mod_base = OTHER; note = 2'-O-methylcytidine
  modified_base 7..8: mod_base = OTHER; note = 2'-O-methyladenosine
  modified_base 9: mod_base = OTHER; note = 2'-fluoroguanosine
  modified_base 10: mod_base = OTHER; note = 2'-fluorocytidine
  modified_base 11: mod_base = OTHER; note = 2'-fluorouridine
  modified_base 12: mod_base = OTHER; note = 2'-O-methyluridine
  modified_base 13..14: mod_base = OTHER; note = 2'-O-methylguanosine
  modified_base 15: mod_base = OTHER; note = 2'-O-methyluridine
  modified_base 16: mod_base = OTHER; note = 2'-O-methylcytidine
  modified_base 17: mod_base = OTHER; note = 2'-O-methyladenosine
  modified_base 18: mod_base = OTHER; note = 2'-O-methyluridine
  modified_base 19: mod_base = OTHER; note = 2'-O-methylcytidine
  modified_base 20: mod_base = OTHER; note = 2'-O-methyluridine
  modified_base 21: mod_base = OTHER; note = 2'-O-methyladenosine
  modified_base 1..2: mod_base = OTHER; note = phosphorothioate linkage
  modified_base 2..3: mod_base = OTHER; note = phosphorothioate linkage
cctgccaagcttggtcatcta

SEQ ID NO: 52 - RNA, 21 nt, synthetic construct
  source 1..21: mol_type = other RNA
  modified_base 1..2: mod_base = OTHER; note = 2'-O-methylcytidine
  modified_base 3: mod_base = OTHER; note = 2'-O-methyluridine
  modified_base 4: mod_base = OTHER; note = 2'-O-methylguanosine
  modified_base 5..6: mod_base = OTHER; note = 2'-O-methylcytidine
  modified_base 7..8: mod_base = OTHER; note = 2'-O-methyladenosine
  modified_base 9: mod_base = OTHER; note = 2'-fluoroguanosine
  modified_base 10: mod_base = OTHER; note = 2'-fluorocytidine
  modified_base 11: mod_base = OTHER; note = 2'-fluorouridine
  modified_base 12: mod_base = OTHER; note = 2'-O-methyluridine
  modified_base 13..14: mod_base = OTHER; note = 2'-O-methylguanosine
  modified_base 15: mod_base = OTHER; note = 2'-O-methyluridine
  modified_base 16: mod_base = OTHER; note = 2'-O-methylcytidine
  modified_base 17: mod_base = OTHER; note = n is R
  modified_base 18: mod_base = OTHER; note = 2'-O-methyluridine
  modified_base 19: mod_base = OTHER; note = 2'-O-methylcytidine
  modified_base 20: mod_base = OTHER; note = 2'-O-methyluridine
  modified_base 21: mod_base = OTHER; note = 2'-O-methyladenosine
  modified_base 1..2: mod_base = OTHER; note = phosphorothioate linkage
  modified_base 2..3: mod_base = OTHER; note = phosphorothioate linkage
cctgccaagcttggtcntcta

SEQ ID NO: 53 - RNA, 21 nt, synthetic construct
  source 1..21: mol_type = other RNA
  modified_base 1: mod_base = OTHER; note = 2'-O-methylcytidine
  modified_base 2: mod_base = OTHER; note = 2'-O-methyluridine
  modified_base 3: mod_base = OTHER; note = 2'-O-methyluridine
  modified_base 4: mod_base = OTHER; note = 2'-O-methylguanosine
  modified_base 5..6: mod_base = OTHER; note = 2'-O-methylcytidine
  modified_base 7..8: mod_base = OTHER; note = 2'-O-methyladenosine
  modified_base 9: mod_base = OTHER; note = 2'-fluoroguanosine
  modified_base 10: mod_base = OTHER; note = 2'-fluorocytidine
  modified_base 11: mod_base = OTHER; note = 2'-fluorouridine
  modified_base 12: mod_base = OTHER; note = 2'-O-methyluridine
  modified_base 13..14: mod_base = OTHER; note = 2'-O-methylguanosine
  modified_base 15: mod_base = OTHER; note = 2'-O-methyluridine
  modified_base 16: mod_base = OTHER; note = 2'-O-methylcytidine
  modified_base 17: mod_base = OTHER; note = 2'-O-methyladenosine
  modified_base 18: mod_base = OTHER; note = 2'-O-methyluridine
  modified_base 19: mod_base = OTHER; note = 2'-O-methylcytidine
  modified_base 20: mod_base = OTHER; note = 2'-O-methyluridine
  modified_base 21: mod_base = OTHER; note = 2'-O-methyladenosine
  modified_base 1..2: mod_base = OTHER; note = phosphorothioate linkage
  modified_base 2..3: mod_base = OTHER; note = phosphorothioate linkage
cttgccaagcttggtcatcta

SEQ ID NO: 54 - RNA, 21 nt, synthetic construct
  source 1..21: mol_type = other RNA
  modified_base 1: mod_base = OTHER; note = 2'-O-methylcytidine
  modified_base 2: mod_base = OTHER; note = 2'-O-methyladenosine
  modified_base 3: mod_base = OTHER; note = 2'-O-methylguanosine
  modified_base 4..5: mod_base = OTHER; note = 2'-O-methylcytidine
  modified_base 6..7: mod_base = OTHER; note = 2'-fluorocytidine
  modified_base 8: mod_base = OTHER; note = 2'-O-methyluridine
  modified_base 9: mod_base = OTHER; note = 2'-fluorouridine
  modified_base 10: mod_base = OTHER; note = 2'-fluoroadenosine
  modified_base 11: mod_base = OTHER; note = 2'-fluorouridine
  modified_base 12: mod_base = OTHER; note = 2'-O-methyluridine
  modified_base 13: mod_base = OTHER; note = 2'-O-methylguanosine
  modified_base 14..15: mod_base = OTHER; note = 2'-O-methyluridine
  modified_base 16: mod_base = OTHER; note = 2'-O-methyladenosine
  modified_base 17: mod_base = OTHER; note = 2'-O-methyluridine
  modified_base 18: mod_base = OTHER; note = 2'-O-methyladenosine
  modified_base 19: mod_base = OTHER; note = 2'-O-methylcytidine
  modified_base 20: mod_base = OTHER; note = 2'-O-methylguanosine
  modified_base 21: mod_base = OTHER; note = 2'-O-methyladenosine
  modified_base 1..2: mod_base = OTHER; note = phosphorothioate linkage
  modified_base 2..3: mod_base = OTHER; note = phosphorothioate linkage
cagccccttattgttatacga

SEQ ID NO: 55 - RNA, 21 nt, synthetic construct
  source 1..21: mol_type = other RNA
  modified_base 1: mod_base = OTHER; note = 2'-O-methylcytidine, linked via a phosphorothioate group
  modified_base 2: mod_base = OTHER; note = n is R
  modified_base 3: mod_base = OTHER; note = 2'-O-methylguanosine
  modified_base 4..7: mod_base = OTHER; note = 2'-O-methylcytidine
  modified_base 8: mod_base = OTHER; note = 2'-O-methyluridine
  modified_base 9: mod_base = OTHER; note = 2'-fluorouridine
  modified_base 10: mod_base = OTHER; note = 2'-fluoroadenosine
  modified_base 1: mod_base = OTHER; note = 2'-O-methylcytidine
  modified_base 12: mod_base = OTHER; note = 2'-O-methyluridine
  modified_base 13: mod_base = OTHER; note = 2'-O-methylguanosine
  modified_base 14..15: mod_base = OTHER; note = 2'-O-methyluridine
  modified_base 16: mod_base = OTHER; note = 2'-O-methyladenosine
  modified_base 17: mod_base = OTHER; note = 2'-O-methyluridine
  modified_base 18: mod_base = OTHER; note = 2'-O-methyladenosine
  modified_base 19: mod_base = OTHER; note = 2'-O-methylcytidine
  modified_base 20: mod_base = OTHER; note = 2'-O-methylguanosine
  modified_base 21: mod_base = OTHER; note = 2'-O-methyladenosine
  modified_base 1..2: mod_base = OTHER; note = phosphorothioate linkage
  modified_base 2..3: mod_base = OTHER; note = phosphorothioate linkage
cngccccttattgttatacga

SEQ ID NO: 56 - RNA, 28 nt, synthetic construct
  source 1..28: mol_type = other RNA
  modified_base 1: mod_base = OTHER; note = 2'-O-methyladenosine
  modified_base 2: mod_base = OTHER; note = 2'-O-methyluridine
  modified_base 3: mod_base = OTHER; note = 2'-O-methylcytidine
  modified_base 6: mod_base = OTHER; note = 2'-O-methyluridine
  modified_base 7: mod_base = OTHER; note = 2'-fluorocytidine
  modified_base 8: mod_base = OTHER; note = 2'-O-methylguanosine
  modified_base 9: mod_base = OTHER; note = 2'-fluorouridine
  modified_base 10: mod_base = OTHER; note = 2'-O-methyladenosine
  modified_base 11: mod_base = OTHER; note = n is Z
  modified_base 12..13: mod_base = OTHER; note = 2'-O-methyladenosine
  modified_base 14: mod_base = OTHER; note = 2'-O-methylcytidine
  modified_base 15..16: mod_base = OTHER; note = 2'-O-methyladenosine
  modified_base 17: mod_base = OTHER; note = 2'-fluorouridine
  modified_base 18: mod_base = OTHER; note = 2'-O-methyladenosine
  modified_base 19: mod_base = OTHER; note = 2'-fluoroadenosine
  modified_base 20: mod_base = OTHER; note = 2'-O-methylguanosine
  modified_base 21: mod_base = OTHER; note = 2'-fluoroguanosine
  modified_base 22: mod_base = OTHER; note = 2'-O-methylguanosine
  modified_base 23: mod_base = OTHER; note = 2'-fluoroguanosine
  modified_base 24: mod_base = OTHER; note = 2'-O-methylcytidine
  modified_base 25: mod_base = OTHER; note = 2'-fluorouridine
  modified_base 26: mod_base = OTHER; note = 2'-O-methylguanosine
  modified_base 27: mod_base = OTHER; note = 2'-O-methyluridine
  modified_base 28: mod_base = OTHER; note = 2'-O-methyluridine
  modified_base 1..2: mod_base = OTHER; note = phosphorothioate linkage
  modified_base 6..7: mod_base = OTHER; note = phosphorothioate linkage
  modified_base 7..8: mod_base = OTHER; note = phosphorothioate linkage
  modified_base 26..27: mod_base = OTHER; note = phosphorothioate linkage
  modified_base 27..28: mod_base = OTHER; note = phosphorothioate linkage
atccctcgtanaacaataaggggctgtt

SEQ ID NO: 57 - RNA, 23 nt, synthetic construct
  source 1..23: mol_type = other RNA
  modified_base 1: mod_base = OTHER; note = E-type vinylphosphonate-modified 2'-O-methyluridine
  modified_base 2: mod_base = OTHER; note = 2'-fluorocytidine
  modified_base 3: mod_base = OTHER; note = 2'-O-methylguanosine
  modified_base 4: mod_base = OTHER; note = 2'-fluorouridine
  modified_base 5: mod_base = OTHER; note = 2'-O-methyladenosine
  modified_base 6: mod_base = OTHER; note = n is Z
  modified_base 7..8: mod_base = OTHER; note = 2'-O-methyladenosine
  modified_base 9: mod_base = OTHER; note = 2'-O-methylcytidine
  modified_base 10..11: mod_base = OTHER; note = 2'-O-methyladenosine
  modified_base 12: mod_base = OTHER; note = 2'-fluorouridine
  modified_base 13: mod_base = OTHER; note = 2'-O-methyladenosine
  modified_base 14: mod_base = OTHER; note = 2'-fluoroadenosine
  modified_base 15: mod_base = OTHER; note = 2'-O-methylguanosine
  modified_base 16: mod_base = OTHER; note = 2'-fluoroguanosine
  modified_base 17: mod_base = OTHER; note = 2'-O-methylguanosine
  modified_base 18: mod_base = OTHER; note = 2'-fluoroguanosine
  modified_base 19: mod_base = OTHER; note = 2'-O-methylcytidine
  modified_base 20: mod_base = OTHER; note = 2'-fluorouridine
  modified_base 21: mod_base = OTHER; note = 2'-O-methylguanosine
  modified_base 22: mod_base = OTHER; note = 2'-O-methyluridine
  modified_base 23: mod_base = OTHER; note = 2'-O-methyluridine
  modified_base 1..2: mod_base = OTHER; note = phosphorothioate linkage
  modified_base 2..3: mod_base = OTHER; note = phosphorothioate linkage
  modified_base 21..22: mod_base = OTHER; note = phosphorothioate linkage
  modified_base 22..23: mod_base = OTHER; note = phosphorothioate linkage
tcgtanaacaataaggggctgtt

SEQ ID NO: 58 - RNA, 23 nt, synthetic construct
  source 1..23: mol_type = other RNA
  modified_base 1: mod_base = OTHER; note = 2'-O-methyluridine
  modified_base 2: mod_base = OTHER; note = 2'-fluorocytidine
  modified_base 3: mod_base = OTHER; note = 2'-O-methylguanosine
  modified_base 4: mod_base = OTHER; note = 2'-fluorouridine
  modified_base 5: mod_base = OTHER; note = 2'-O-methyladenosine
  modified_base 6: mod_base = OTHER; note = n is Z
  modified_base 7..8: mod_base = OTHER; note = 2'-O-methyladenosine
  modified_base 9: mod_base = OTHER; note = 2'-O-methylcytidine
  modified_base 10..11: mod_base = OTHER; note = 2'-O-methyladenosine
  modified_base 12: mod_base = OTHER; note = 2'-fluorouridine
  modified_base 13: mod_base = OTHER; note = 2'-O-methyladenosine
  modified_base 14: mod_base = OTHER; note = 2'-fluoroadenosine
  modified_base 15: mod_base = OTHER; note = 2'-O-methylguanosine
  modified_base 16: mod_base = OTHER; note = 2'-fluoroguanosine
  modified_base 17: mod_base = OTHER; note = 2'-O-methylguanosine
  modified_base 18: mod_base = OTHER; note = 2'-fluoroguanosine
  modified_base 19: mod_base = OTHER; note = 2'-O-methylcytidine
  modified_base 20: mod_base = OTHER; note = 2'-fluorouridine
  modified_base 21: mod_base = OTHER; note = 2'-O-methylguanosine
  modified_base 22: mod_base = OTHER; note = 2'-O-methyluridine
  modified_base 23: mod_base = OTHER; note = 2'-O-methyluridine
  modified_base 1..2: mod_base = OTHER; note = phosphorothioate linkage
  modified_base 2..3: mod_base = OTHER; note = phosphorothioate linkage
  modified_base 21..22: mod_base = OTHER; note = phosphorothioate linkage
  modified_base 22..23: mod_base = OTHER; note = phosphorothioate linkage
tcgtanaacaataaggggctgtt

SEQ ID NO: 59 - RNA, 28 nt, synthetic construct
  source 1..28: mol_type = other RNA
  modified_base 1: mod_base = OTHER; note = 2'-O-methyladenosine
  modified_base 2: mod_base = OTHER; note = 2'-O-methyluridine
  modified_base 3: mod_base = OTHER; note = 2'-O-methylcytidine
  modified_base 6: mod_base = OTHER; note = 2'-O-methyluridine
  modified_base 7: mod_base = OTHER; note = 2'-fluorocytidine
  modified_base 8: mod_base = OTHER; note = 2'-O-methylguanosine
  modified_base 9: mod_base = OTHER; note = 2'-fluorouridine
  modified_base 10: mod_base = OTHER; note = 2'-O-methyladenosine
  modified_base 11: mod_base = OTHER; note = n is Z
  modified_base 12..13: mod_base = OTHER; note = 2'-O-methyladenosine
  modified_base 14: mod_base = OTHER; note = 2'-O-methylcytidine
  modified_base 15..16: mod_base = OTHER; note = 2'-O-methyladenosine
  modified_base 17: mod_base = OTHER; note = 2'-fluorouridine
  modified_base 18: mod_base = OTHER; note = 2'-O-methyladenosine
  modified_base 19: mod_base = OTHER; note = 2'-fluoroadenosine
  modified_base 20: mod_base = OTHER; note = 2'-O-methylguanosine
  modified_base 21: mod_base = OTHER; note = 2'-fluoroguanosine
  modified_base 22: mod_base = OTHER; note = 2'-O-methylguanosine
  modified_base 23: mod_base = OTHER; note = 2'-fluoroguanosine
  modified_base 24: mod_base = OTHER; note = 2'-O-methylcytidine
  modified_base 25: mod_base = OTHER; note = 2'-fluorouridine
  modified_base 26: mod_base = OTHER; note = 2'-O-methylguanosine
  modified_base 27: mod_base = OTHER; note = 2'-O-methylcytidine
  modified_base 28: mod_base = OTHER; note = 2'-O-methylcytidine
  modified_base 1..2: mod_base = OTHER; note = phosphorothioate linkage
  modified_base 6..7: mod_base = OTHER; note = phosphorothioate linkage
  modified_base 7..8: mod_base = OTHER; note = phosphorothioate linkage
  modified_base 26..27: mod_base = OTHER; note = phosphorothioate linkage
  modified_base 27..28: mod_base = OTHER; note = phosphorothioate linkage
atccctcgtanaacaataaggggctgcc

SEQ ID NO: 60 - RNA, 26 nt, synthetic construct
  source 1..26: mol_type = other RNA
  modified_base 1: mod_base = OTHER; note = 2'-O-methyladenosine
  modified_base 2: mod_base = OTHER; note = 2'-O-methyluridine
  modified_base 3: mod_base = OTHER; note = 2'-O-methylcytidine
  modified_base 6: mod_base = OTHER; note = 2'-O-methyluridine
  modified_base 7: mod_base = OTHER; note = 2'-fluorocytidine
  modified_base 8: mod_base = OTHER; note = 2'-O-methylguanosine
  modified_base 9: mod_base = OTHER; note = 2'-fluorouridine
  modified_base 10: mod_base = OTHER; note = 2'-O-methyladenosine
  modified_base 11: mod_base = OTHER; note = n is Z
  modified_base 12..13: mod_base = OTHER; note = 2'-O-methyladenosine
  modified_base 14: mod_base = OTHER; note = 2'-O-methylcytidine
  modified_base 15..16: mod_base = OTHER; note = 2'-O-methyladenosine
  modified_base 17: mod_base = OTHER; note = 2'-fluorouridine
  modified_base 18: mod_base = OTHER; note = 2'-O-methyladenosine
  modified_base 19: mod_base = OTHER; note = 2'-fluoroadenosine
  modified_base 20: mod_base = OTHER; note = 2'-O-methylguanosine
  modified_base 21: mod_base = OTHER; note = 2'-fluoroguanosine
  modified_base 22: mod_base = OTHER; note = 2'-O-methylguanosine
  modified_base 23: mod_base = OTHER; note = 2'-fluoroguanosine
  modified_base 24: mod_base = OTHER; note = 2'-O-methylcytidine
  modified_base 25: mod_base = OTHER; note = 2'-fluorouridine
  modified_base 26: mod_base = OTHER; note = 2'-O-methylguanosine
  modified_base 1..2: mod_base = OTHER; note = phosphorothioate linkage
  modified_base 6..7: mod_base = OTHER; note = phosphorothioate linkage
  modified_base 7..8: mod_base = OTHER; note = phosphorothioate linkage
  modified_base 24..25: mod_base = OTHER; note = phosphorothioate linkage
  modified_base 25..26: mod_base = OTHER; note = phosphorothioate linkage
atccctcgtanaacaataaggggctg

SEQ ID NO: 61 - RNA, 28 nt, synthetic construct
  source 1..28: mol_type = other RNA
  modified_base 1: mod_base = OTHER; note = 2'-O-methyladenosine
  modified_base 2: mod_base = OTHER; note = 2'-O-methyluridine
  modified_base 3..4: mod_base = OTHER; note = 2'-O-methylcytidine
  modified_base 6: mod_base = OTHER; note = 2'-O-methyluridine
  modified_base 7: mod_base = OTHER; note = 2'-fluorocytidine
  modified_base 8: mod_base = OTHER; note = 2'-O-methylguanosine
  modified_base 9: mod_base = OTHER; note = 2'-fluorouridine
  modified_base 10: mod_base = OTHER; note = 2'-O-methyladenosine
  modified_base 11: mod_base = OTHER; note = n is Z
  modified_base 12..13: mod_base = OTHER; note = 2'-O-methyladenosine
  modified_base 14: mod_base = OTHER; note = 2'-O-methylcytidine
  modified_base 15..16: mod_base = OTHER; note = 2'-O-methyladenosine
  modified_base 17: mod_base = OTHER; note = 2'-fluorouridine
  modified_base 18: mod_base = OTHER; note = 2'-O-methyladenosine
  modified_base 19: mod_base = OTHER; note = 2'-fluoroadenosine
  modified_base 20: mod_base = OTHER; note = 2'-O-methylguanosine
  modified_base 21: mod_base = OTHER; note = 2'-fluoroguanosine
  modified_base 22: mod_base = OTHER; note = 2'-O-methylguanosine
  modified_base 23: mod_base = OTHER; note = 2'-fluoroguanosine
  modified_base 24: mod_base = OTHER; note = 2'-O-methylcytidine
  modified_base 25: mod_base = OTHER; note = 2'-fluorouridine
  modified_base 26: mod_base = OTHER; note = 2'-O-methylguanosine
  modified_base 27: mod_base = OTHER; note = 2'-O-methyluridine
  modified_base 28: mod_base = OTHER; note = 2'-O-methyluridine
  modified_base 1..2: mod_base = OTHER; note = phosphorothioate linkage
  modified_base 6..7: mod_base = OTHER; note = phosphorothioate linkage
  modified_base 7..8: mod_base = OTHER; note = phosphorothioate linkage
  modified_base 26..27: mod_base = OTHER; note = phosphorothioate linkage
  modified_base 27..28: mod_base = OTHER; note = phosphorothioate linkage
atccctcgtanaacaataaggggctgtt

SEQ ID NO: 62 - RNA, 28 nt, synthetic construct
  source 1..28: mol_type = other RNA
  modified_base 1: mod_base = OTHER; note = 2'-O-methyladenosine
  modified_base 2: mod_base = OTHER; note = 2'-O-methyluridine
  modified_base 3..4: mod_base = OTHER; note = 2'-O-methylcytidine
  modified_base 6: mod_base = OTHER; note = 2'-O-methyluridine
  modified_base 7: mod_base = OTHER; note = 2'-fluorocytidine
  modified_base 8: mod_base = OTHER; note = 2'-O-methylguanosine
  modified_base 9: mod_base = OTHER; note = 2'-fluorouridine
  modified_base 10: mod_base = OTHER; note = 2'-O-methyladenosine
  modified_base 11: mod_base = OTHER; note = n is Z
  modified_base 12..13: mod_base = OTHER; note = 2'-O-methyladenosine
  modified_base 14: mod_base = OTHER; note = 2'-O-methylcytidine
  modified_base 15..16: mod_base = OTHER; note = 2'-O-methyladenosine
  modified_base 17: mod_base = OTHER; note = 2'-O-methyluridine
  modified_base 18: mod_base = OTHER; note = 2'-O-methyladenosine
  modified_base 19: mod_base = OTHER; note = 2'-fluoroadenosine
  modified_base 20: mod_base = OTHER; note = 2'-O-methylguanosine
  modified_base 21: mod_base = OTHER; note = 2'-fluoroguanosine
  modified_base 22: mod_base = OTHER; note = 2'-O-methylguanosine
  modified_base 23: mod_base = OTHER; note = 2'-fluoroguanosine
  modified_base 24: mod_base = OTHER; note = 2'-O-methylcytidine
  modified_base 25: mod_base = OTHER; note = 2'-fluorouridine
  modified_base 26: mod_base = OTHER; note = 2'-O-methylguanosine
  modified_base 27: mod_base = OTHER; note = 2'-O-methyluridine
  modified_base 28: mod_base = OTHER; note = 2'-O-methyluridine
  modified_base 1..2: mod_base = OTHER; note = phosphorothioate linkage
  modified_base 2..3: mod_base = OTHER; note = phosphorothioate linkage
  modified_base 6..7: mod_base = OTHER; note = phosphorothioate linkage
  modified_base 7..8: mod_base = OTHER; note = phosphorothioate linkage
  modified_base 26..27: mod_base = OTHER; note = phosphorothioate linkage
  modified_base 27..28: mod_base = OTHER; note = phosphorothioate linkage
atccctcgtanaacaataaggggctgtt

SEQ ID NO: 63 - RNA, 26 nt, synthetic construct
  source 1..26: mol_type = other RNA
  modified_base 1: mod_base = OTHER; note = 2'-O-methyladenosine
  modified_base 2: mod_base = OTHER; note = 2'-O-methyluridine
  modified_base 3..4: mod_base = OTHER; note = 2'-O-methylcytidine
  modified_base 6: mod_base = OTHER; note = 2'-O-methyluridine
  modified_base 7: mod_base = OTHER; note = 2'-fluorocytidine
  modified_base 8: mod_base = OTHER; note = 2'-O-methylguanosine
  modified_base 9: mod_base = OTHER; note = 2'-fluorouridine
  modified_base 10: mod_base = OTHER; note = 2'-O-methyladenosine
  modified_base 11: mod_base = OTHER; note = n is Z
  modified_base 12..13: mod_base = OTHER; note = 2'-O-methyladenosine
  modified_base 14: mod_base = OTHER; note = 2'-O-methylcytidine
  modified_base 15..16: mod_base = OTHER; note = 2'-O-methyladenosine
  modified_base 17: mod_base = OTHER; note = 2'-fluorouridine
  modified_base 18: mod_base = OTHER; note = 2'-O-methyladenosine
  modified_base 19: mod_base = OTHER; note = 2'-fluoroadenosine
  modified_base 20: mod_base = OTHER; note = 2'-O-methylguanosine
  modified_base 21: mod_base = OTHER; note = 2'-fluoroguanosine
  modified_base 22: mod_base = OTHER; note = 2'-O-methylguanosine
  modified_base 23: mod_base = OTHER; note = 2'-fluoroguanosine
  modified_base 24: mod_base = OTHER; note = 2'-O-methylcytidine
  modified_base 25: mod_base = OTHER; note = 2'-fluorouridine
  modified_base 26: mod_base = OTHER; note = 2'-O-methylguanosine
  modified_base 1..2: mod_base = OTHER; note = phosphorothioate linkage
  modified_base 6..7: mod_base = OTHER; note = phosphorothioate linkage
  modified_base 7..8: mod_base = OTHER; note = phosphorothioate linkage
  modified_base 24..25: mod_base = OTHER; note = phosphorothioate linkage
  modified_base 25..26: mod_base = OTHER; note = phosphorothioate linkage
atccctcgtanaacaataaggggctg

SEQ ID NO: 64 - RNA, 25 nt, synthetic construct
  source 1..25: mol_type = other RNA
  modified_base 1: mod_base = OTHER; note = 2'-O-methyluridine
  modified_base 3: mod_base = OTHER; note = 2'-O-methyluridine
  modified_base 4: mod_base = OTHER; note = 2'-fluorocytidine
  modified_base 5: mod_base = OTHER; note = 2'-O-methylguanosine
  modified_base 6: mod_base = OTHER; note = 2'-fluorouridine
  modified_base 7: mod_base = OTHER; note = 2'-O-methyladenosine
  modified_base 8: mod_base = OTHER; note = n is Z
  modified_base 9..10: mod_base = OTHER; note = 2'-O-methyladenosine
  modified_base 11: mod_base = OTHER; note = 2'-O-methylcytidine
  modified_base 12..13: mod_base = OTHER; note = 2'-O-methyladenosine
  modified_base 14: mod_base = OTHER; note = 2'-fluorouridine
  modified_base 15: mod_base = OTHER; note = 2'-O-methyladenosine
  modified_base 16: mod_base = OTHER; note = 2'-fluoroadenosine
  modified_base 17: mod_base = OTHER; note = 2'-O-methylguanosine
  modified_base 18: mod_base = OTHER; note = 2'-fluoroguanosine
  modified_base 19: mod_base = OTHER; note = 2'-O-methylguanosine
  modified_base 20: mod_base = OTHER; note = 2'-fluoroguanosine
  modified_base 21: mod_base = OTHER; note = 2'-O-methylcytidine
  modified_base 22: mod_base = OTHER; note = 2'-fluorouridine
  modified_base 23: mod_base = OTHER; note = 2'-O-methylguanosine
  modified_base 24: mod_base = OTHER; note = 2'-O-methyluridine
  modified_base 25: mod_base = OTHER; note = 2'-O-methyluridine
  modified_base 3..4: mod_base = OTHER; note = phosphorothioate linkage
  modified_base 4..5: mod_base = OTHER; note = phosphorothioate linkage
  modified_base 23..24: mod_base = OTHER; note = phosphorothioate linkage
  modified_base 24..25: mod_base = OTHER; note = phosphorothioate linkage
tctcgtanaacaataaggggctgtt

SEQ ID NO: 65 - RNA, 23 nt, synthetic construct
  source 1..23: mol_type = other RNA
  modified_base 1: mod_base = OTHER; note = 2'-O-methyluridine
  modified_base 3: mod_base = OTHER; note = 2'-O-methyluridine
  modified_base 4: mod_base = OTHER; note = 2'-fluorocytidine
  modified_base 5: mod_base = OTHER; note = 2'-O-methylguanosine
  modified_base 6: mod_base = OTHER; note = 2'-O-methyluridine
  modified_base 7: mod_base = OTHER; note = 2'-O-methyladenosine
  modified_base 8: mod_base = OTHER; note = 2'-fluorouridine
  modified_base 9: mod_base = OTHER; note = n is R
  modified_base 10: mod_base = OTHER; note = 2'-O-methyladenosine
  modified_base 11: mod_base = OTHER; note = 2'-O-methylcytidine
  modified_base 12..13: mod_base = OTHER; note = 2'-O-methyladenosine
  modified_base 14: mod_base = OTHER; note = 2'-O-methyluridine
  modified_base 15: mod_base = OTHER; note = 2'-O-methyladenosine
  modified_base 16: mod_base = OTHER; note = 2'-fluoroadenosine
  modified_base 17: mod_base = OTHER; note = 2'-O-methylguanosine
  modified_base 18: mod_base = OTHER; note = 2'-fluoroguanosine
  modified_base 19..20: mod_base = OTHER; note = 2'-O-methylguanosine
  modified_base 21: mod_base = OTHER; note = 2'-O-methylcytidine
  modified_base 22: mod_base = OTHER; note = 2'-O-methyluridine
  modified_base 23: mod_base = OTHER; note = 2'-O-methyluridine
  modified_base 3..4: mod_base = OTHER; note = phosphorothioate linkage
  modified_base 4..5: mod_base = OTHER; note = phosphorothioate linkage
  modified_base 21..22: mod_base = OTHER; note = phosphorothioate linkage
  modified_base 22..23: mod_base = OTHER; note = phosphorothioate linkage
tctcgtatnacaataaggggctt

SEQ ID NO: 66 - RNA, 23 nt, synthetic construct
  source 1..23: mol_type = other RNA
  modified_base 1: mod_base = OTHER; note = 2'-O-methyluridine
  modified_base 3: mod_base = OTHER; note = 2'-O-methyluridine
  modified_base 4: mod_base = OTHER; note = 2'-fluorocytidine
  modified_base 5: mod_base = OTHER; note = 2'-O-methylguanosine
  modified_base 6: mod_base = OTHER; note = 2'-fluorouridine
  modified_base 7: mod_base = OTHER; note = 2'-O-methyladenosine
  modified_base 8: mod_base = OTHER; note = 2'-fluorouridine
  modified_base 9: mod_base = OTHER; note = n is R
  modified_base 10: mod_base = OTHER; note = 2'-O-methyladenosine
  modified_base 11: mod_base = OTHER; note = 2'-O-methylcytidine
  modified_base 12..13: mod_base = OTHER; note = 2'-O-methyladenosine
  modified_base 14: mod_base = OTHER; note = 2'-O-methyluridine
  modified_base 15: mod_base = OTHER; note = 2'-O-methyladenosine
  modified_base 16: mod_base = OTHER; note = 2'-fluoroguanosine
  modified_base 17: mod_base = OTHER; note = 2'-O-methylguanosine
  modified_base 18: mod_base = OTHER; note = 2'-fluoroguanosine
  modified_base 19: mod_base = OTHER; note = 2'-O-methylguanosine
  modified_base 20: mod_base = OTHER; note = 2'-fluoroguanosine
  modified_base 21: mod_base = OTHER; note = 2'-O-methylcytidine
  modified_base 22: mod_base = OTHER; note = 2'-fluorouridine
  modified_base 23: mod_base = OTHER; note = 2'-O-methylguanosine
  modified_base 3..4: mod_base = OTHER; note = phosphorothioate linkage
  modified_base 4..5: mod_base = OTHER; note = phosphorothioate linkage
  modified_base 21..22: mod_base = OTHER; note = phosphorothioate linkage
  modified_base 22..23: mod_base = OTHER; note = phosphorothioate linkage
tctcgtatnacaataaggggctg

SEQ ID NO: 67 - RNA, 21 nt, synthetic construct
  source 1..21: mol_type = other RNA
  modified_base 1: mod_base = OTHER; note = 2'-O-methyluridine
  modified_base 2: mod_base = OTHER; note = 2'-fluoroadenosine
  modified_base 3: mod_base = OTHER; note = 2'-O-methylguanosine
  modified_base 4: mod_base = OTHER; note = 2'-O-methyladenosine
  modified_base 5: mod_base = OTHER; note = 2'-O-methyluridine
  modified_base 6: mod_base = OTHER; note = n is R
  modified_base 7: mod_base = OTHER; note = 2'-fluoroadenosine
  modified_base 8..9: mod_base = OTHER; note = 2'-O-methylcytidine
  modified_base 10..11: mod_base = OTHER; note = 2'-O-methyladenosine
  modified_base 12: mod_base = OTHER; note = 2'-O-methylguanosine
  modified_base 13: mod_base = OTHER; note = 2'-fluorocytidine
  modified_base 14: mod_base = OTHER; note = 2'-O-methyluridine
  modified_base 15: mod_base = OTHER; note = 2'-fluorouridine
  modified_base 16..17: mod_base = OTHER; note = 2'-O-methylguanosine
  modified_base 18: mod_base = OTHER; note = 2'-O-methylcytidine
  modified_base 19: mod_base = OTHER; note = 2'-O-methyladenosine
  modified_base 20: mod_base = OTHER; note = n is R
  modified_base 21: mod_base = OTHER; note = 2'-O-methylguanosine
  modified_base 1..2: mod_base = OTHER; note = phosphorothioate linkage
  modified_base 2..3: mod_base = OTHER; note = phosphorothioate linkage
  modified_base 19..20: mod_base = OTHER; note = phosphorothioate linkage
  modified_base 20..21: mod_base = OTHER; note = phosphorothioate linkage
tagatnaccaagcttggcang

SEQ ID NO: 68 - RNA, 21 nt, synthetic construct
  source 1..21: mol_type = other RNA
  modified_base 1: mod_base = OTHER; note = 2'-O-methyluridine
  modified_base 2: mod_base = OTHER; note = 2'-fluoroadenosine
  modified_base 3: mod_base = OTHER; note = 2'-O-methylguanosine
  modified_base 4: mod_base = OTHER; note = 2'-O-methyladenosine
  modified_base 5: mod_base = OTHER; note = 2'-O-methyluridine
  modified_base 6: mod_base = OTHER; note = n is R
  modified_base 7: mod_base = OTHER; note = 2'-fluoroadenosine
  modified_base 8..9: mod_base = OTHER; note = 2'-O-methylcytidine
  modified_base 10..11: mod_base = OTHER; note = 2'-O-methyladenosine
  modified_base 12: mod_base = OTHER; note = 2'-O-methylguanosine
  modified_base 13: mod_base = OTHER; note = 2'-O-methylcytidine
  modified_base 14: mod_base = OTHER; note = 2'-fluorouridine
  modified_base 15: mod_base = OTHER; note = 2'-O-methyluridine
  modified_base 16: mod_base = OTHER; note = 2'-fluoroguanosine
  modified_base 17: mod_base = OTHER; note = 2'-O-methylguanosine
  modified_base 18: mod_base = OTHER; note = 2'-O-methylcytidine
  modified_base 19: mod_base = OTHER; note = 2'-O-methyladenosine
  modified_base 20: mod_base = OTHER; note = n is R
  modified_base 21: mod_base = OTHER; note = 2'-O-methylguanosine
  modified_base 1..2: mod_base = OTHER; note = phosphorothioate linkage
  modified_base 2..3: mod_base = OTHER; note = phosphorothioate linkage
  modified_base 19..20: mod_base = OTHER; note = phosphorothioate linkage
  modified_base 20..21: mod_base = OTHER; note = phosphorothioate linkage
tagatnaccaagcttggcang

SEQ ID NO: 69 - RNA, 22 nt, synthetic construct
  source 1..22: mol_type = other RNA
  modified_base 1: mod_base = OTHER; note = 2'-O-methyluridine
  modified_base 2: mod_base = OTHER; note = 2'-fluoroadenosine
  modified_base 3: mod_base = OTHER; note = 2'-fluoroguanosine
  modified_base 4: mod_base = OTHER; note = 2'-fluoroadenosine
  modified_base 5: mod_base = OTHER; note = 2'-fluorouridine
  modified_base 6: mod_base = OTHER; note = n is R
  modified_base 7: mod_base = OTHER; note = 2'-fluoroadenosine
  modified_base 8..9: mod_base = OTHER; note = 2'-O-methylcytidine
  modified_base 10: mod_base = OTHER; note = 2'-fluoroadenosine
  modified_base 11: mod_base = OTHER; note = 2'-O-methyladenosine
  modified_base 12: mod_base = OTHER; note = 2'-O-methylguanosine
  modified_base 13: mod_base = OTHER; note = 2'-O-methylcytidine
  modified_base 14: mod_base = OTHER; note = 2'-fluorouridine
  modified_base 15: mod_base = OTHER; note = 2'-O-methyluridine
  modified_base 16..17: mod_base = OTHER; note = 2'-O-methylguanosine
  modified_base 18: mod_base = OTHER; note = 2'-O-methylcytidine
  modified_base 19: mod_base = OTHER; note = 2'-O-methyladenosine
  modified_base 20: mod_base = OTHER; note = n is R
  modified_base 21: mod_base = OTHER; note = 2'-O-methylguanosine
  modified_base 22: mod_base = OTHER; note = 2'-O-methylguanosine
  modified_base 1..2: mod_base = OTHER; note = phosphorothioate linkage
  modified_base 2..3: mod_base = OTHER; note = phosphorothioate linkage
  modified_base 3..4: mod_base = OTHER; note = phosphorothioate linkage
  modified_base 20..21: mod_base = OTHER; note = phosphorothioate linkage
  modified_base 21..22: mod_base = OTHER; note = phosphorothioate linkage
tagatnaccaagcttggcangg

SEQ ID NO: 70 - RNA, 23 nt, synthetic construct
  source 1..23: mol_type = other RNA
  modified_base 1: mod_base = OTHER; note = 2'-O-methyluridine
  modified_base 3: mod_base = OTHER; note = 2'-O-methyluridine
  modified_base 4: mod_base = OTHER; note = 2'-fluorocytidine
  modified_base 5: mod_base = OTHER; note = 2'-O-methylguanosine
  modified_base 6: mod_base = OTHER; note = 2'-fluorouridine
  modified_base 7: mod_base = OTHER; note = 2'-O-methyladenosine
  modified_base 8: mod_base = OTHER; note = 2'-fluorouridine
  modified_base 9: mod_base = OTHER; note = n is Z
  modified_base 10: mod_base = OTHER; note = 2'-O-methyladenosine
  modified_base 11: mod_base = OTHER; note = 2'-O-methylcytidine
  modified_base 12..13: mod_base = OTHER; note = 2'-O-methyladenosine
  modified_base 14: mod_base = OTHER; note = 2'-fluorouridine
  modified_base 15: mod_base = OTHER; note = 2'-O-methyladenosine
  modified_base 16: mod_base = OTHER; note = 2'-fluoroadenosine
  modified_base 17: mod_base = OTHER; note = 2'-O-methylguanosine
  modified_base 18: mod_base = OTHER; note = 2'-fluoroguanosine
  modified_base 19: mod_base = OTHER; note = 2'-O-methylguanosine
  modified_base 20: mod_base = OTHER; note = 2'-fluoroguanosine
  modified_base 21: mod_base = OTHER; note = 2'-O-methylcytidine
  modified_base 22: mod_base = OTHER; note = 2'-fluorouridine
  modified_base 23: mod_base = OTHER; note = 2'-O-methylguanosine
  modified_base 3..4: mod_base = OTHER; note = phosphorothioate linkage
  modified_base 4..5: mod_base = OTHER; note = phosphorothioate linkage
  modified_base 21..22: mod_base = OTHER; note = phosphorothioate linkage
  modified_base 22..23: mod_base = OTHER; note = phosphorothioate linkage
tctcgtatnacaataaggggctg

SEQ ID NO: 71 - RNA, 22 nt, synthetic construct
  source 1..22: mol_type = other RNA
  modified_base 1: mod_base = OTHER; note = E-type vinylphosphonate-modified 2'-O-methyluridine
  modified_base 2: mod_base = OTHER; note = 2'-fluorocytidine
  modified_base 3: mod_base = OTHER; note = 2'-O-methylguanosine
  modified_base 4: mod_base = OTHER; note = 2'-O-methyluridine
  modified_base 5: mod_base = OTHER; note = 2'-O-methyladenosine
  modified_base 6: mod_base = OTHER; note = 2'-fluorouridine
  modified_base 7: mod_base = OTHER; note = n is R
  modified_base 8: mod_base = OTHER; note = 2'-O-methyladenosine
  modified_base 9: mod_base = OTHER; note = 2'-O-methylcytidine
  modified_base 10..11: mod_base = OTHER; note = 2'-O-methyladenosine
  modified_base 12: mod_base = OTHER; note = 2'-fluorouridine
  modified_base 13: mod_base = OTHER; note = 2'-O-methyladenosine
  modified_base 14: mod_base = OTHER; note = 2'-fluoroadenosine
  modified_base 15: mod_base = OTHER; note = 2'-O-methylguanosine
  modified_base 16: mod_base = OTHER; note = 2'-fluoroguanosine
  modified_base 17: mod_base = OTHER; note = 2'-O-methylguanosine
  modified_base 18: mod_base = OTHER; note = 2'-fluoroguanosine
  modified_base 19: mod_base = OTHER; note = 2'-O-methylcytidine
  modified_base 20: mod_base = OTHER; note = 2'-fluorouridine
  modified_base 21: mod_base = OTHER; note = 2'-O-methylguanosine
  modified_base 1..2: mod_base = OTHER; note = phosphorothioate linkage
  modified_base 2..3: mod_base = OTHER; note = phosphorothioate linkage
  modified_base 19..20: mod_base = OTHER; note = phosphorothioate linkage
  modified_base 20..21: mod_base = OTHER; note = phosphorothioate linkage
tcgtatnacaataaggggctgt

SEQ ID NO: 72 - RNA, 22 nt, synthetic construct
  source 1..22: mol_type = other RNA
  modified_base 1: mod_base = OTHER; note = E-type vinylphosphonate-modified 2'-O-methyluridine
  modified_base 2: mod_base = OTHER; note = 2'-fluorocytidine
  modified_base 3: mod_base = OTHER; note = 2'-O-methylguanosine
  modified_base 4: mod_base = OTHER; note = 2'-fluorouridine
  modified_base 5: mod_base = OTHER; note = 2'-O-methyladenosine
  modified_base 6: mod_base = OTHER; note = 2'-fluorouridine
  modified_base 7: mod_base = OTHER; note = n is Z
  modified_base 8: mod_base = OTHER; note = 2'-O-methyladenosine
  modified_base 9: mod_base = OTHER; note = 2'-O-methylcytidine
  modified_base 10..11: mod_base = OTHER; note = 2'-O-methyladenosine
  modified_base 12: mod_base = OTHER; note = 2'-fluorouridine
  modified_base 13: mod_base = OTHER; note = 2'-O-methyladenosine
  modified_base 14: mod_base = OTHER; note = 2'-fluoroadenosine
  modified_base 15: mod_base = OTHER; note = 2'-O-methylguanosine
  modified_base 16: mod_base = OTHER; note = 2'-fluoroguanosine
  modified_base 17: mod_base = OTHER; note = 2'-O-methylguanosine
  modified_base 18: mod_base = OTHER; note = 2'-fluoroguanosine
  modified_base 19: mod_base = OTHER; note = 2'-O-methylcytidine
  modified_base 20: mod_base = OTHER; note = 2'-fluorouridine
  modified_base 21: mod_base = OTHER; note = 2'-O-methylguanosine
  modified_base 1..2: mod_base = OTHER; note = phosphorothioate linkage
  modified_base 2..3: mod_base = OTHER; note = phosphorothioate linkage
  modified_base 19..20: mod_base = OTHER; note = phosphorothioate linkage
  modified_base 20..21: mod_base = OTHER; note = phosphorothioate linkage
tcgtatnacaataaggggctgt

SEQ ID NO: 73 - RNA, 23 nt, synthetic construct
  source 1..23: mol_type = other RNA
  modified_base 1: mod_base = OTHER; note = E-type vinylphosphonate-modified 2'-O-methyluridine
  modified_base 2: mod_base = OTHER; note = 2'-fluorocytidine
  modified_base 3: mod_base = OTHER; note = 2'-O-methylguanosine
  modified_base 4: mod_base = OTHER; note = 2'-O-methyluridine
  modified_base 5: mod_base = OTHER; note = 2'-O-methyladenosine
  modified_base 6: mod_base = OTHER; note = 2'-fluorouridine
  modified_base 7: mod_base = OTHER; note = n is R
  modified_base 8: mod_base = OTHER; note = 2'-O-methyladenosine
  modified_base 9: mod_base = OTHER; note = 2'-O-methylcytidine
  modified_base 10..11: mod_base = OTHER; note = 2'-O-methyladenosine
  modified_base 12: mod_base = OTHER; note = 2'-O-methyluridine
  modified_base 13: mod_base = OTHER; note = 2'-O-methyladenosine
  modified_base 14: mod_base = OTHER; note = 2'-fluoroadenosine
  modified_base 15: mod_base = OTHER; note = 2'-O-methylguanosine
  modified_base 16: mod_base = OTHER; note = 2'-fluoroguanosine
  modified_base 17..18: mod_base = OTHER; note = 2'-O-methylguanosine
  modified_base 19: mod_base = OTHER; note = 2'-O-methylcytidine
  modified_base 20: mod_base = OTHER; note = n is R
  modified_base 21: mod_base = OTHER; note = 2'-O-methylguanosine
  modified_base 22: mod_base = OTHER; note = 2'-O-methyluridine
  modified_base 23: mod_base = OTHER; note = 2'-O-methyluridine
  modified_base 1..2: mod_base = OTHER; note = phosphorothioate linkage
  modified_base 2..3: mod_base = OTHER; note = phosphorothioate linkage
  modified_base 21..22: mod_base = OTHER; note = phosphorothioate linkage
  modified_base 22..23: mod_base = OTHER; note = phosphorothioate linkage
tcgtatnacaataaggggcngtt

SEQ ID NO: 74 - RNA, 23 nt, synthetic construct
  source 1..23: mol_type = other RNA
  modified_base 1: mod_base = OTHER; note = E-type vinylphosphonate-modified 2'-O-methyluridine
  modified_base 2: mod_base = OTHER; note = 2'-deoxycytidine
  modified_base 3: mod_base = OTHER; note = 2'-O-methylguanosine
  modified_base 4: mod_base = OTHER; note = 2'-O-methyluridine
  modified_base 5: mod_base = OTHER; note = 2'-deoxyadenosine
  modified_base 6: mod_base = OTHER; note = 2'-O-methyluridine
  modified_base 7: mod_base = OTHER; note = n is 2'-deoxy-R
  modified_base 8: mod_base = OTHER; note = 2'-O-methyladenosine
  modified_base 9: mod_base = OTHER; note = 2'-O-methylcytidine
  modified_base 10..11: mod_base = OTHER; note = 2'-O-methyladenosine
  modified_base 12: mod_base = OTHER; note = 2'-deoxythymidine
  modified_base 13: mod_base = OTHER; note = 2'-O-methyladenosine
  modified_base 14: mod_base = OTHER; note = 2'-fluoroadenosine
  modified_base 15: mod_base = OTHER; note = 2'-O-methylguanosine
  modified_base 16: mod_base = OTHER; note = 2'-fluoroguanosine
  modified_base 17..18: mod_base = OTHER; note = 2'-O-methylguanosine
  modified_base 19: mod_base = OTHER; note = 2'-O-methylcytidine
  modified_base 20: mod_base = OTHER; note = n is R
  modified_base 21: mod_base = OTHER; note = 2'-O-methylguanosine
  modified_base 22: mod_base = OTHER; note = 2'-O-methyluridine
  modified_base 23: mod_base = OTHER; note = 2'-O-methyluridine
  modified_base 1..2: mod_base = OTHER; note = phosphorothioate linkage
  modified_base 2..3: mod_base = OTHER; note = phosphorothioate linkage
  modified_base 21..22: mod_base = OTHER; note = phosphorothioate linkage
  modified_base 22..23: mod_base = OTHER; note = phosphorothioate linkage
tcgtatnacaataaggggcngtt

SEQ ID NO: 75 - RNA, 23 nt, synthetic construct
  source 1..23: mol_type = other RNA
  modified_base 1: mod_base = OTHER; note = E-type vinylphosphonate-modified 2'-O-methyluridine
  modified_base 2: mod_base = OTHER; note = 2'-fluoroadenosine
  modified_base 3: mod_base = OTHER; note = 2'-O-methylguanosine
  modified_base 4: mod_base = OTHER; note = 2'-O-methyladenosine
  modified_base 5: mod_base = OTHER; note = 2'-O-methyluridine
  modified_base 6: mod_base = OTHER; note = 2'-fluoroguanosine
  modified_base 7: mod_base = OTHER; note = n is R
  modified_base 8..9: mod_base = OTHER; note = 2'-O-methylcytidine
  modified_base 10..11: mod_base = OTHER; note = 2'-O-methyladenosine
  modified_base 12: mod_base = OTHER; note = 2'-O-methylguanosine
  modified_base 13: mod_base = OTHER; note = 2'-O-methylcytidine
  modified_base 14: mod_base = OTHER; note = 2'-fluorouridine
  modified_base 15: mod_base = OTHER; note = 2'-O-methyluridine
  modified_base 16: mod_base = OTHER; note = 2'-fluoroguanosine
  modified_base 17: mod_base = OTHER; note = 2'-O-methylguanosine
  modified_base 18: mod_base = OTHER; note = 2'-O-methylcytidine
  modified_base 19: mod_base = OTHER; note = n is R
  modified_base 20: mod_base = OTHER; note = 2'-O-methylguanosine
  modified_base 21: mod_base = OTHER; note = 2'-O-methylguanosine
  modified_base 22: mod_base = OTHER; note = 2'-O-methyluridine
  modified_base 23: mod_base = OTHER; note = 2'-O-methyluridine
  modified_base 1..2: mod_base = OTHER; note = phosphorothioate linkage
  modified_base 2..3: mod_base = OTHER; note = phosphorothioate linkage
  modified_base 21..22: mod_base = OTHER; note = phosphorothioate linkage
  modified_base 22..23: mod_base = OTHER; note = phosphorothioate linkage
tagatgnccaagcttggcnggtt

SEQ ID NO: 76 - RNA, 23 nt, synthetic construct
  source 1..23: mol_type = other RNA
  modified_base 1: mod_base = OTHER; note = E-type vinylphosphonate-modified 2'-O-methyluridine
  modified_base 2: mod_base = OTHER; note = 2'-deoxyadenosine
  modified_base 3: mod_base = OTHER; note = 2'-O-methylguanosine
  modified_base 4: mod_base = OTHER; note = 2'-O-methyladenosine
  modified_base 5: mod_base = OTHER; note = 2'-deoxythymidine
  modified_base 6: mod_base = OTHER; note = 2'-O-methylguanosine
  modified_base 7: mod_base = OTHER; note = n is 2'-deoxy-R
  modified_base 8..9: mod_base = OTHER; note = 2'-O-methylcytidine
  modified_base 10..11: mod_base = OTHER; note = 2'-O-methyladenosine
  modified_base 12: mod_base = OTHER; note = 2'-deoxyguanosine
  modified_base 13: mod_base = OTHER; note = 2'-O-methylcytidine
  modified_base 14: mod_base = OTHER; note = 2'-fluorouridine
  modified_base 15: mod_base = OTHER; note = 2'-O-methyluridine
  modified_base 16: mod_base = OTHER; note = 2'-fluoroguanosine
  modified_base 17: mod_base = OTHER; note = 2'-O-methylguanosine
  modified_base 18: mod_base = OTHER; note = 2'-O-methylcytidine
  modified_base 19: mod_base = OTHER; note = n is R
  modified_base 20: mod_base = OTHER; note = 2'-O-methylguanosine
  modified_base 21: mod_base = OTHER; note = 2'-O-methylguanosine
  modified_base 22: mod_base = OTHER; note = 2'-O-methyluridine
  modified_base 23: mod_base = OTHER; note = 2'-O-methyluridine
  modified_base 1..2: mod_base = OTHER; note = phosphorothioate linkage
  modified_base 2..3: mod_base = OTHER; note = phosphorothioate linkage
  modified_base 21..22: mod_base = OTHER; note = phosphorothioate linkage
  modified_base 22..23: mod_base = OTHER; note = phosphorothioate linkage
tagatgnccaagcttggcnggtt

SEQ ID NO: 77 - RNA, 23 nt, synthetic construct
  source 1..23: mol_type = other RNA
  modified_base 1: mod_base = OTHER; note = n is mDVPU
  modified_base 2: mod_base = OTHER; note = 2'-deoxycytidine
  modified_base 3: mod_base = OTHER; note = 2'-O-methylguanosine
  modified_base 4: mod_base = OTHER; note = 2'-O-methyluridine
  modified_base 5: mod_base = OTHER; note = 2'-deoxyadenosine
  modified_base 6: mod_base = OTHER; note = 2'-O-methyluridine
  modified_base 7: mod_base = OTHER; note = n is 2'-deoxy-R
  modified_base 8: mod_base = OTHER; note = 2'-O-methyladenosine
  modified_base 9: mod_base = OTHER; note = 2'-O-methylcytidine
  modified_base 10..11: mod_base = OTHER; note = 2'-O-methyladenosine
  modified_base 12: mod_base = OTHER; note = 2'-deoxythymidine
  modified_base 13: mod_base = OTHER; note = 2'-O-methyladenosine
  modified_base 14: mod_base = OTHER; note = 2'-fluoroadenosine
  modified_base 15: mod_base = OTHER; note = 2'-O-methylguanosine
  modified_base 16: mod_base = OTHER; note = 2'-fluoroguanosine
  modified_base 17..18: mod_base = OTHER; note = 2'-O-methylguanosine
  modified_base 19: mod_base = OTHER; note = 2'-O-methylcytidine
  modified_base 20: mod_base = OTHER; note = n is R
  modified_base 21: mod_base = OTHER; note = 2'-O-methylguanosine
  modified_base 22: mod_base = OTHER; note = 2'-O-methyluridine
  modified_base 23: mod_base = OTHER; note = 2'-O-methyluridine
  modified_base 1..2: mod_base = OTHER; note = phosphorothioate linkage
  modified_base 2..3: mod_base = OTHER; note = phosphorothioate linkage
  modified_base 21..22: mod_base = OTHER; note = phosphorothioate linkage
  modified_base 22..23: mod_base = OTHER; note = phosphorothioate linkage
ncgtatnacaataaggggcngtt

SEQ ID NO: 78 - RNA, 23 nt, synthetic construct
  source 1..23: mol_type = other RNA
  modified_base 1: mod_base = OTHER; note = 2'-O-methyluridine
  modified_base 3: mod_base = OTHER; note = 2'-O-methyluridine
  modified_base 4: mod_base = OTHER; note = 2'-fluoroadenosine
  modified_base 5: mod_base = OTHER; note = 2'-O-methylguanosine
  modified_base 6: mod_base = OTHER; note = 2'-fluoroadenosine
  modified_base 7: mod_base = OTHER; note = 2'-O-methyluridine
  modified_base 8: mod_base = OTHER; note = 2'-fluoroguanosine
  modified_base 9: mod_base = OTHER; note = n is R
  modified_base 10..11: mod_base = OTHER; note = 2'-O-methylcytidine
  modified_base 12..13: mod_base = OTHER; note = 2'-O-methyladenosine
  modified_base 14: mod_base = OTHER; note = 2'-fluoroguanosine
  modified_base 15: mod_base = OTHER; note = 2'-O-methylcytidine
  modified_base 16: mod_base = OTHER; note = 2'-fluorouridine
  modified_base 17: mod_base = OTHER; note = 2'-O-methyluridine
  modified_base 18: mod_base = OTHER; note = 2'-fluoroguanosine
  modified_base 19: mod_base = OTHER; note = 2'-O-methylguanosine
  modified_base 20: mod_base = OTHER; note = 2'-fluorocytidine
  modified_base 21: mod_base = OTHER; note = n is R
  modified_base 22: mod_base = OTHER; note = 2'-fluoroguanosine
  modified_base 23: mod_base = OTHER; note = 2'-O-methylguanosine
  modified_base 3..4: mod_base = OTHER; note = phosphorothioate linkage
  modified_base 4..5: mod_base = OTHER; note = phosphorothioate linkage
  modified_base 21..22: mod_base = OTHER; note = phosphorothioate linkage
  modified_base 22..23: mod_base = OTHER; note = phosphorothioate linkage
tctagatgnccaagcttggcngg

SEQ ID NO: 79 - RNA, 23 nt, synthetic construct
  source 1..23: mol_type = other RNA
  modified_base 1: mod_base = OTHER; note = n is B29
  modified_base 2: mod_base = OTHER; note = 2'-deoxycytidine
  modified_base 3: mod_base = OTHER; note = 2'-O-methylguanosine
  modified_base 4: mod_base = OTHER; note = 2'-O-methyluridine
  modified_base 5: mod_base = OTHER; note = 2'-deoxyadenosine
  modified_base 6: mod_base = OTHER; note = 2'-O-methyluridine
  modified_base 7: mod_base = OTHER; note = n is 2'-deoxy-R
  modified_base 8: mod_base = OTHER; note = 2'-O-methyladenosine
  modified_base 9: mod_base = OTHER; note = 2'-O-methylcytidine
  modified_base 10..11: mod_base = OTHER; note = 2'-O-methyladenosine
  modified_base 12: mod_base = OTHER; note = 2'-deoxythymidine
  modified_base 13: mod_base = OTHER; note = 2'-O-methyladenosine
  modified_base 14: mod_base = OTHER; note = 2'-fluoroadenosine
  modified_base 15: mod_base = OTHER; note = 2'-O-methylguanosine
  modified_base 16: mod_base = OTHER; note = 2'-fluoroguanosine
  modified_base 17..18: mod_base = OTHER; note = 2'-O-methylguanosine
  modified_base 19: mod_base = OTHER; note = 2'-O-methylcytidine
  modified_base 20: mod_base = OTHER; note = n is R
  modified_base 21: mod_base = OTHER; note = 2'-O-methylguanosine
  modified_base 22: mod_base = OTHER; note = 2'-O-methyluridine
  modified_base 23: mod_base = OTHER; note = 2'-O-methyluridine
  modified_base 1..2: mod_base = OTHER; note = phosphorothioate linkage
  modified_base 2..3: mod_base = OTHER; note = phosphorothioate linkage
  modified_base 21..22: mod_base = OTHER; note = phosphorothioate linkage
  modified_base 22..23: mod_base = OTHER; note = phosphorothioate linkage
ncgtatnacaataaggggcngtt

SEQ ID NO: 80 - RNA, 23 nt, synthetic construct
  source 1..23: mol_type = other RNA
  modified_base 1: mod_base = OTHER; note = n is B33
  modified_base 2: mod_base = OTHER; note = 2'-deoxycytidine
  modified_base 3: mod_base = OTHER; note = 2'-O-methylguanosine
  modified_base 4: mod_base = OTHER; note = 2'-O-methyluridine
  modified_base 5: mod_base = OTHER; note = 2'-deoxyadenosine
  modified_base 6: mod_base = OTHER; note = 2'-O-methyluridine
  modified_base 7: mod_base = OTHER; note = n is 2'-deoxy-R
  modified_base 8: mod_base = OTHER; note = 2'-O-methyladenosine
  modified_base 9: mod_base = OTHER; note = 2'-O-methylcytidine
  modified_base 10..11: mod_base = OTHER; note = 2'-O-methyladenosine
  modified_base 12: mod_base = OTHER; note = 2'-deoxythymidine
  modified_base 13: mod_base = OTHER; note = 2'-O-methyladenosine
  modified_base 14: mod_base = OTHER; note = 2'-fluoroadenosine
  modified_base 15: mod_base = OTHER; note = 2'-O-methylguanosine
  modified_base 16: mod_base = OTHER; note = 2'-fluoroguanosine
  modified_base 17..18: mod_base = OTHER; note = 2'-O-methylguanosine
  modified_base 19: mod_base = OTHER; note = 2'-O-methylcytidine
  modified_base 20: mod_base = OTHER; note = n is R
  modified_base 21: mod_base = OTHER; note = 2'-O-methylguanosine
  modified_base 22: mod_base = OTHER; note = 2'-O-methyluridine
  modified_base 23: mod_base = OTHER; note = 2'-O-methyluridine
  modified_base 1..2: mod_base = OTHER; note = phosphorothioate linkage
  modified_base 2..3: mod_base = OTHER; note = phosphorothioate linkage
  modified_base 21..22: mod_base = OTHER; note = phosphorothioate linkage
  modified_base 22..23: mod_base = OTHER; note = phosphorothioate linkage
ncgtatnacaataaggggcngtt

SEQ ID NO: 81 - RNA, 23 nt, synthetic construct
  source 1..23: mol_type = other RNA
  modified_base 1: mod_base = OTHER; note = n is B30
  modified_base 2: mod_base = OTHER; note = 2'-deoxycytidine
  modified_base 3: mod_base = OTHER; note = 2'-O-methylguanosine
  modified_base 4: mod_base = OTHER; note = 2'-O-methyluridine
  modified_base 5: mod_base = OTHER; note = 2'-deoxyadenosine
  modified_base 6: mod_base = OTHER; note = 2'-O-methyluridine
  modified_base 7: mod_base = OTHER; note = n is 2'-deoxy-R
  modified_base 8: mod_base = OTHER; note = 2'-O-methyladenosine
  modified_base 9: mod_base = OTHER; note = 2'-O-methylcytidine
  modified_base 10..11: mod_base = OTHER; note = 2'-O-methyladenosine
  modified_base 12: mod_base = OTHER; note = 2'-deoxythymidine
  modified_base 13: mod_base = OTHER; note = 2'-O-methyladenosine
  modified_base 14: mod_base = OTHER; note = 2'-fluoroadenosine
  modified_base 15: mod_base = OTHER; note = 2'-O-methylguanosine
  modified_base 16: mod_base = OTHER; note = 2'-fluoroguanosine
  modified_base 17..18: mod_base = OTHER; note = 2'-O-methylguanosine
  modified_base 19: mod_base = OTHER; note = 2'-O-methylcytidine
  modified_base 20: mod_base = OTHER; note = n is R
  modified_base 21: mod_base = OTHER; note = 2'-O-methylguanosine
  modified_base 22: mod_base = OTHER; note = 2'-O-methyluridine
  modified_base 23: mod_base = OTHER; note = 2'-O-methyluridine
  modified_base 1..2: mod_base = OTHER; note = phosphorothioate linkage
  modified_base 2..3: mod_base = OTHER; note = phosphorothioate linkage
  modified_base 21..22: mod_base = OTHER; note = phosphorothioate linkage
  modified_base 22..23: mod_base = OTHER; note = phosphorothioate linkage
ncgtatnacaataaggggcngtt

SEQ ID NO: 82 - RNA, 23 nt, synthetic construct
  source 1..23: mol_type = other RNA
  modified_base 1: mod_base = OTHER; note = n is mDVPU
  modified_base 2: mod_base = OTHER; note = 2'-deoxyadenosine
  modified_base 3: mod_base = OTHER; note = 2'-O-methylguanosine
  modified_base 4: mod_base = OTHER; note = 2'-O-methyladenosine
  modified_base 5: mod_base = OTHER; note = 2'-deoxythymidine
  modified_base 6: mod_base = OTHER; note = 2'-O-methylguanosine
  modified_base 7: mod_base = OTHER; note = n is 2'-deoxy-R
  modified_base 8..9: mod_base = OTHER; note = 2'-O-methylcytidine
  modified_base 10..11: mod_base = OTHER; note = 2'-deoxyguanosine
  modified_base 13: mod_base = OTHER; note = 2'-O-methylcytidine
  modified_base 14: mod_base = OTHER; note = 2'-fluorouridine
  modified_base 15: mod_base = OTHER; note = 2'-O-methyluridine
  modified_base 16: mod_base = OTHER; note = 2'-fluoroguanosine
  modified_base 17: mod_base = OTHER; note = 2'-O-methylguanosine
  modified_base 18: mod_base = OTHER; note = 2'-O-methylcytidine
  modified_base 19: mod_base = OTHER; note = n is R
  modified_base 20: mod_base = OTHER; note = 2'-O-methylguanosine
  modified_base 21: mod_base = OTHER; note = 2'-O-methylguanosine
  modified_base 22: mod_base = OTHER; note = 2'-O-methyluridine
  modified_base 23: mod_base = OTHER; note = 2'-O-methyluridine
  modified_base 1..2: mod_base = OTHER; note = phosphorothioate linkage
  modified_base 2..3: mod_base = OTHER; note = phosphorothioate linkage
  modified_base 21..22: mod_base = OTHER; note = phosphorothioate linkage
  modified_base 22..23: mod_base = OTHER; note = phosphorothioate linkage
nagatgnccaagcttggcnggtt

SEQ ID NO: 83 - RNA, 23 nt, synthetic construct
  source 1..23: mol_type = other RNA
  modified_base 1: mod_base = OTHER; note = n is B33
  modified_base 2: mod_base = OTHER; note = 2'-deoxyadenosine
  modified_base 3: mod_base = OTHER; note = 2'-O-methylguanosine
  modified_base 4: mod_base = OTHER; note = 2'-O-methyladenosine
  modified_base 5: mod_base = OTHER; note = 2'-deoxythymidine
  modified_base 6: mod_base = OTHER; note = 2'-O-methylguanosine
  modified_base 7: mod_base = OTHER; note = n is 2'-deoxy-R
  modified_base 8..9: mod_base = OTHER; note = 2'-O-methylcytidine
  modified_base 10..11: mod_base = OTHER; note = 2'-O-methyladenosine
  modified_base 12: mod_base = OTHER; note = 2'-deoxyguanosine
  modified_base 13: mod_base = OTHER; note = 2'-O-methylcytidine
  modified_base 14: mod_base = OTHER; note = 2'-fluorouridine
  modified_base 15: mod_base = OTHER; note = 2'-O-methyluridine
  modified_base 16: mod_base = OTHER; note = 2'-fluoroguanosine
  modified_base 17: mod_base = OTHER; note = 2'-O-methylguanosine
  modified_base 18: mod_base = OTHER; note = 2'-O-methylcytidine
  modified_base 19: mod_base = OTHER; note = n is R
  modified_base 20: mod_base = OTHER; note = 2'-O-methylguanosine
  modified_base 21: mod_base = OTHER; note = 2'-O-methylguanosine
  modified_base 22: mod_base = OTHER; note = 2'-O-methyluridine
  modified_base 23: mod_base = OTHER; note = 2'-O-methyluridine
  modified_base 1..2: mod_base = OTHER; note = phosphorothioate linkage
  modified_base 2..3: mod_base = OTHER; note = phosphorothioate linkage
  modified_base 21..22: mod_base = OTHER; note = phosphorothioate linkage
  modified_base 22..23: mod_base = OTHER; note = phosphorothioate linkage
nagatgnccaagcttggcnggtt

SEQ ID NO: 84 - RNA, 23 nt, synthetic construct
  source 1..23: mol_type = other RNA
  modified_base 1: mod_base = OTHER; note = n is B34
  modified_base 2: mod_base = OTHER; note = 2'-deoxyadenosine
  modified_base 3: mod_base = OTHER; note = 2'-O-methylguanosine
  modified_base 4: mod_base = OTHER; note = 2'-O-methyladenosine
  modified_base 5: mod_base = OTHER; note = 2'-deoxythymidine
  modified_base 6: mod_base = OTHER; note = 2'-O-methylguanosine
  modified_base 7: mod_base = OTHER; note = n is 2'-deoxy-R
  modified_base 8..9: mod_base = OTHER; note = 2'-O-methylcytidine
  modified_base 10..11: mod_base = OTHER; note = 2'-O-methyladenosine
  modified_base 12: mod_base = OTHER; note = 2'-deoxyguanosine
  modified_base 13: mod_base = OTHER; note = 2'-O-methylcytidine
  modified_base 14: mod_base = OTHER; note = 2'-fluorouridine
  modified_base 15: mod_base = OTHER; note = 2'-O-methyluridine
  modified_base 16: mod_base = OTHER; note = 2'-fluoroguanosine
  modified_base 17: mod_base = OTHER; note = 2'-O-methylguanosine
  modified_base 18: mod_base = OTHER; note = 2'-O-methylcytidine
  modified_base 19: mod_base = OTHER; note = n is R
  modified_base 20: mod_base = OTHER; note = 2'-O-methylguanosine
  modified_base 21: mod_base = OTHER; note = 2'-O-methylguanosine
  modified_base 22: mod_base = OTHER; note = 2'-O-methyluridine
  modified_base 23: mod_base = OTHER; note = 2'-O-methyluridine
  modified_base 1..2: mod_base = OTHER; note = phosphorothioate linkage
  modified_base 2..3: mod_base = OTHER; note = phosphorothioate linkage
  modified_base 21..22: mod_base = OTHER; note = phosphorothioate linkage
  modified_base 22..23: mod_base = OTHER; note = phosphorothioate linkage
nagatgnccaagcttggcnggtt

SEQ ID NO: 85 - RNA, 23 nt, synthetic construct
  source 1..23: mol_type = other RNA
  modified_base 1: mod_base = OTHER; note = n is B36
  modified_base 2: mod_base = OTHER; note = 2'-deoxyadenosine
  modified_base 3: mod_base = OTHER; note = 2'-O-methylguanosine
  modified_base 4: mod_base = OTHER; note = 2'-O-methyladenosine
  modified_base 5: mod_base = OTHER; note = 2'-deoxythymidine
  modified_base 6: mod_base = OTHER; note = 2'-O-methylguanosine
  modified_base 7: mod_base = OTHER; note = n is 2'-deoxy-R
  modified_base 8..9: mod_base = OTHER; note = 2'-O-methylcytidine
  modified_base 10..11: mod_base = OTHER; note = 2'-O-methyladenosine
  modified_base 12: mod_base = OTHER; note = 2'-deoxyguanosine
  modified_base 13: mod_base = OTHER; note = 2'-O-methylcytidine
  modified_base 14: mod_base = OTHER; note = 2'-fluorouridine
  modified_base 15: mod_base = OTHER; note = 2'-O-methyluridine
  modified_base 16: mod_base = OTHER; note = 2'-fluoroguanosine
  modified_base 17: mod_base = OTHER; note = 2'-O-methylguanosine
  modified_base 18: mod_base = OTHER; note = 2'-O-methylcytidine
  modified_base 19: mod_base = OTHER; note = n is R
  modified_base 20: mod_base = OTHER; note = 2'-O-methylguanosine
  modified_base 21: mod_base = OTHER; note = 2'-O-methylguanosine
  modified_base 22: mod_base = OTHER; note = 2'-O-methyluridine
  modified_base 23: mod_base = OTHER; note = 2'-O-methyluridine
  modified_base 1..2: mod_base = OTHER; note = phosphorothioate linkage
  modified_base 2..3: mod_base = OTHER; note = phosphorothioate linkage
  modified_base 21..22: mod_base = OTHER; note = phosphorothioate linkage
  modified_base 22..23: mod_base = OTHER; note = phosphorothioate linkage
nagatgnccaagcttggcnggtt

SEQ ID NO: 86 - RNA, 23 nt, synthetic construct
  source 1..23: mol_type = other RNA
  modified_base 1: mod_base = OTHER; note = 2'-O-methyluridine
  modified_base 3: mod_base = OTHER; note = 2'-O-methyluridine
  modified_base 4: mod_base = OTHER; note = 2'-fluoroadenosine
  modified_base 5: mod_base = OTHER; note = 2'-O-methylguanosine
  modified_base 6: mod_base = OTHER; note = 2'-fluoroadenosine
  modified_base 7: mod_base = OTHER; note = 2'-O-methyluridine
  modified_base 8: mod_base = OTHER; note = n is R
  modified_base 9: mod_base = OTHER; note = 2'-O-methyladenosine
  modified_base 10..11: mod_base = OTHER; note = 2'-O-methylcytidine
  modified_base 12..13: mod_base = OTHER; note = 2'-O-methyladenosine
  modified_base 14: mod_base = OTHER; note = 2'-fluoroguanosine
  modified_base 15: mod_base = OTHER; note = 2'-O-methylcytidine
  modified_base 16: mod_base = OTHER; note = 2'-fluorouridine
  modified_base 17: mod_base = OTHER; note = 2'-O-methyluridine
  modified_base 18: mod_base = OTHER; note = 2'-fluoroguanosine
  modified_base 19: mod_base = OTHER; note = 2'-O-methylguanosine
  modified_base 20: mod_base = OTHER; note = 2'-O-methylcytidine
  modified_base 21: mod_base = OTHER; note = 2'-O-methyladenosine
  modified_base 22: mod_base = OTHER; note = 2'-fluoroguanosine
  modified_base 23: mod_base = OTHER; note = 2'-O-methylguanosine
  modified_base 3..4: mod_base = OTHER; note = phosphorothioate linkage
  modified_base 4..5: mod_base = OTHER; note = phosphorothioate linkage
  modified_base 21..22: mod_base = OTHER; note = phosphorothioate linkage
  modified_base 22..23: mod_base = OTHER; note = phosphorothioate linkage
tctagatnaccaagcttggcagg

SEQ ID NO: 87 - RNA, 23 nt, synthetic construct
  source 1..23: mol_type = other RNA
  modified_base 1: mod_base = OTHER; note = 2'-O-methyluridine
  modified_base 2: mod_base = OTHER; note = 2'-deoxycytidine
  modified_base 3: mod_base = OTHER; note = 2'-O-methylguanosine
  modified_base 4: mod_base = OTHER; note = 2'-O-methyluridine
  modified_base 5: mod_base = OTHER; note = 2'-deoxyadenosine
  modified_base 6: mod_base = OTHER; note = 2'-O-methyluridine
  modified_base 7: mod_base = OTHER; note = n is 2'-deoxy-R
  modified_base 8: mod_base = OTHER; note = 2'-O-methyladenosine
  modified_base 9: mod_base = OTHER; note = 2'-O-methylcytidine
  modified_base 10..11: mod_base = OTHER; note = 2'-O-methyladenosine
  modified_base 12: mod_base = OTHER; note = 2'-deoxythymidine
  modified_base 13: mod_base = OTHER; note = 2'-O-methyladenosine
  modified_base 14: mod_base = OTHER; note = 2'-fluoroadenosine
  modified_base 15: mod_base = OTHER; note = 2'-O-methylguanosine
  modified_base 16: mod_base = OTHER; note = 2'-fluoroguanosine
  modified_base 17..18: mod_base = OTHER; note = 2'-O-methylguanosine
  modified_base 19: mod_base = OTHER; note = 2'-O-methylcytidine
  modified_base 20: mod_base = OTHER; note = n is R
  modified_base 21: mod_base = OTHER; note = 2'-O-methylguanosine
  modified_base 22: mod_base = OTHER; note = 2'-O-methyluridine
  modified_base 23: mod_base = OTHER; note = 2'-O-methyluridine
  modified_base 1..2: mod_base = OTHER; note = phosphorothioate linkage
  modified_base 2..3: mod_base = OTHER; note = phosphorothioate linkage
  modified_base 21..22: mod_base = OTHER; note = phosphorothioate linkage
  modified_base 22..23: mod_base = OTHER; note = phosphorothioate linkage
tcgtatnacaataaggggcngtt

SEQ ID NO: 88 - RNA, 23 nt, synthetic construct
  source 1..23: mol_type = other RNA
  modified_base 1: mod_base = OTHER; note = 2'-O-methyluridine
  modified_base 3: mod_base = OTHER; note = 2'-O-methyluridine
  modified_base 4: mod_base = OTHER; note = 2'-fluoroadenosine
  modified_base 5: mod_base = OTHER; note = 2'-O-methylguanosine
  modified_base 6: mod_base = OTHER; note = 2'-fluoroadenosine
  modified_base 7: mod_base = OTHER; note = 2'-O-methyluridine
  modified_base 8: mod_base = OTHER; note = 2'-fluoroguanosine
  modified_base 9: mod_base = OTHER; note = n is R
  modified_base 10..11: mod_base = OTHER; note = 2'-O-methylcytidine
  modified_base 12..13: mod_base = OTHER; note = 2'-O-methyladenosine
  modified_base 14: mod_base = OTHER; note = 2'-fluoroguanosine
  modified_base 15: mod_base = OTHER; note = 2'-O-methylcytidine
  modified_base 16: mod_base = OTHER; note = 2'-fluorouridine
  modified_base 17: mod_base = OTHER; note = 2'-O-methylguanosine
  modified_base 18: mod_base = OTHER; note = 2'-fluoroguanosine
  modified_base 19: mod_base = OTHER; note = 2'-O-methylguanosine
  modified_base 20: mod_base = OTHER; note = 2'-fluorocytidine
  modified_base 21: mod_base = OTHER; note = 2'-O-methyladenosine
  modified_base 22: mod_base = OTHER; note = 2'-fluoroadenosine, linked via a phosphorothioate group
  modified_base 23: mod_base = OTHER; note = 2'-O-methylguanosine
  modified_base 3..4: mod_base = OTHER; note = phosphorothioate linkage
  modified_base 4..5: mod_base = OTHER; note = phosphorothioate linkage
  modified_base 21..22: mod_base = OTHER; note = phosphorothioate linkage
  modified_base 22..23: mod_base = OTHER; note = phosphorothioate linkage
tctagatgnccaagcttggcaag

SEQ ID NO: 89 - RNA, 23 nt, synthetic construct
  source 1..23: mol_type = other RNA
  modified_base 1: mod_base = OTHER; note = n is B33
  modified_base 2: mod_base = OTHER; note = 2'-deoxycytidine
  modified_base 3: mod_base = OTHER; note = 2'-O-methylguanosine
  modified_base 4: mod_base = OTHER; note = 2'-O-methyluridine
  modified_base 5: mod_base = OTHER; note = 2'-deoxyadenosine
  modified_base 6: mod_base = OTHER; note = 2'-O-methyluridine
  modified_base 7..8: mod_base = OTHER; note = 2'-O-methyladenosine
  modified_base 9: mod_base = OTHER; note = 2'-O-methylcytidine
  modified_base 10..11: mod_base = OTHER; note = 2'-O-methyladenosine
  modified_base 12: mod_base = OTHER; note = 2'-deoxythymidine
  modified_base 13: mod_base = OTHER; note = 2'-O-methyladenosine
  modified_base 14: mod_base = OTHER; note = 2'-fluoroadenosine
  modified_base 15: mod_base = OTHER; note = 2'-O-methylguanosine
  modified_base 16: mod_base = OTHER; note = 2'-fluoroguanosine
  modified_base 17..18: mod_base = OTHER; note = 2'-O-methylguanosine
  modified_base 19: mod_base = OTHER; note = 2'-O-methylcytidine
  modified_base 20: mod_base = OTHER; note = n is R
  modified_base 21: mod_base = OTHER; note = 2'-O-methylguanosine
  modified_base 22: mod_base = OTHER; note = 2'-O-methyluridine
  modified_base 23: mod_base = OTHER; note = 2'-O-methyluridine
  modified_base 1..2: mod_base = OTHER; note = phosphorothioate linkage
  modified_base 2..3: mod_base = OTHER; note = phosphorothioate linkage
  modified_base 21..22: mod_base = OTHER; note = phosphorothioate linkage
  modified_base 22..23: mod_base = OTHER; note = phosphorothioate linkage
ncgtataacaataaggggcngtt

SEQ ID NO: 90 - RNA, 23 nt, synthetic construct
  source 1..23: mol_type = other RNA
  modified_base 1: mod_base = OTHER; note = n is B33
  modified_base 2: mod_base = OTHER; note = 2'-fluorocytidine
  modified_base 3: mod_base = OTHER; note = 2'-O-methylguanosine
  modified_base 4: mod_base = OTHER; note = 2'-O-methyluridine
  modified_base 5: mod_base = OTHER; note = 2'-O-methyladenosine
  modified_base 6: mod_base = OTHER; note = 2'-O-methyluridine
  modified_base 7: mod_base = OTHER; note = n is 2'-deoxy-R
  modified_base 8: mod_base = OTHER; note = 2'-O-methyladenosine
  modified_base 9: mod_base = OTHER; note = 2'-O-methylcytidine
  modified_base 10..11: mod_base = OTHER; note = 2'-O-methyladenosine
  modified_base 12: mod_base = OTHER; note = 2'-deoxythymidine
  modified_base 13: mod_base = OTHER; note = 2'-O-methyladenosine
  modified_base 14: mod_base = OTHER; note = 2'-fluoroadenosine
  modified_base 15: mod_base = OTHER; note = 2'-O-methylguanosine
  modified_base 16: mod_base = OTHER; note = 2'-fluoroguanosine
  modified_base 17..18: mod_base = OTHER; note = 2'-O-methylguanosine
  modified_base 19: mod_base = OTHER; note = 2'-O-methylcytidine
  modified_base 20: mod_base = OTHER; note = n is R
  modified_base 21: mod_base = OTHER; note = 2'-O-methylguanosine
  modified_base 22: mod_base = OTHER; note = 2'-O-methyluridine
  modified_base 23: mod_base = OTHER; note = 2'-O-methyluridine
  modified_base 1..2: mod_base = OTHER; note = phosphorothioate linkage
  modified_base 2..3: mod_base = OTHER; note = phosphorothioate linkage
  modified_base 21..22: mod_base = OTHER; note = phosphorothioate linkage
  modified_base 22..23: mod_base = OTHER; note = phosphorothioate linkage
ncgtatnacaataaggggcngtt

SEQ ID NO: 91 - RNA, 23 nt, synthetic construct
  source 1..23: mol_type = other RNA
  modified_base 1: mod_base = OTHER; note = n is B33
  modified_base 2: mod_base = OTHER; note = 2'-O-methylcytidine
  modified_base 3: mod_base = OTHER; note = 2'-O-methylguanosine
  modified_base 4: mod_base = OTHER; note = 2'-O-methyluridine
  modified_base 5: mod_base = OTHER; note = 2'-deoxyadenosine
  modified_base 6: mod_base = OTHER; note = 2'-O-methyluridine
  modified_base 7: mod_base = OTHER; note = n is 2'-deoxy-R
  modified_base 8: mod_base = OTHER; note = 2'-O-methyladenosine
  modified_base 9: mod_base = OTHER; note = 2'-O-methylcytidine
  modified_base 10..11: mod_base = OTHER; note = 2'-O-methyladenosine
  modified_base 12: mod_base = OTHER; note = 2'-deoxythymidine
  modified_base 13: mod_base = OTHER; note = 2'-O-methyladenosine
  modified_base 14: mod_base = OTHER; note = 2'-fluoroadenosine
  modified_base 15: mod_base = OTHER; note = 2'-O-methylguanosine
  modified_base 16: mod_base = OTHER; note = 2'-fluoroguanosine
  modified_base 17..18: mod_base = OTHER; note = 2'-O-methylguanosine
  modified_base 19: mod_base = OTHER; note = 2'-O-methylcytidine
  modified_base 20: mod_base = OTHER; note = n is R
  modified_base 21: mod_base = OTHER; note = 2'-O-methylguanosine
  modified_base 22: mod_base = OTHER; note = 2'-O-methyluridine
  modified_base 23: mod_base = OTHER; note = 2'-O-methyluridine
  modified_base 1..2: mod_base = OTHER; note = phosphorothioate linkage
  modified_base 2..3: mod_base = OTHER; note = phosphorothioate linkage
  modified_base 21..22: mod_base = OTHER; note = phosphorothioate linkage
  modified_base 22..23: mod_base = OTHER; note = phosphorothioate linkage
ncgtatnacaataaggggcngtt

SEQ ID NO: 92 - RNA, 23 nt, synthetic construct
  source 1..23: mol_type = other RNA
  modified_base 1: mod_base = OTHER; note = 2'-O-methyluridine
  modified_base 3: mod_base = OTHER; note = 2'-O-methyluridine
  modified_base 4: mod_base = OTHER; note = 2'-fluorocytidine
  modified_base 5: mod_base = OTHER; note = 2'-O-methylguanosine
  modified_base 6: mod_base = OTHER; note = 2'-fluorouridine
  modified_base 7: mod_base = OTHER; note = 2'-O-methyladenosine
  modified_base 8: mod_base = OTHER; note = 2'-fluorouridine
  modified_base 9..10: mod_base = OTHER; note = 2'-O-methyladenosine
  modified_base 11: mod_base = OTHER; note = 2'-O-methylcytidine
  modified_base 12..13: mod_base = OTHER; note = 2'-O-methyladenosine
  modified_base 14: mod_base = OTHER; note = 2'-fluorouridine
  modified_base 15: mod_base = OTHER; note = 2'-O-methyladenosine
  modified_base 16: mod_base = OTHER; note = 2'-fluoroadenosine
  modified_base 17: mod_base = OTHER; note = 2'-O-methylguanosine
  modified_base 18: mod_base = OTHER; note = 2'-fluoroguanosine
  modified_base 19: mod_base = OTHER; note = 2'-O-methylguanosine
  modified_base 20: mod_base = OTHER; note = 2'-fluoroguanosine
  modified_base 21: mod_base = OTHER; note = 2'-O-methylcytidine, linked via a phosphorothioate group
  modified_base 22: mod_base = OTHER; note = 2'-fluorouridine
  modified_base 23: mod_base = OTHER; note = 2'-O-methylguanosine
  modified_base 3..4: mod_base = OTHER; note = phosphorothioate linkage
  modified_base 4..5: mod_base = OTHER; note = phosphorothioate linkage
  modified_base 21..22: mod_base = OTHER; note = phosphorothioate linkage
  modified_base 22..23: mod_base = OTHER; note = phosphorothioate linkage
tctcgtataacaataaggggctg

SEQ ID NO: 93 - RNA, 23 nt, synthetic construct
  source 1..23: mol_type = other RNA
  modified_base 1: mod_base = OTHER; note = n is B33
  modified_base 2: mod_base = OTHER; note = 2'-deoxycytidine
  modified_base 3: mod_base = OTHER; note = 2'-O-methylguanosine
  modified_base 4: mod_base = OTHER; note = 2'-O-methyluridine
  modified_base 5: mod_base = OTHER; note = 2'-deoxyadenosine
  modified_base 6: mod_base = OTHER; note = 2'-O-methyluridine
  modified_base 7: mod_base = OTHER; note = n is 2'-deoxy-R
  modified_base 8: mod_base = OTHER; note = 2'-O-methyladenosine
  modified_base 9: mod_base = OTHER; note = 2'-O-methylcytidine
  modified_base 10..11: mod_base = OTHER; note = 2'-O-methyladenosine
  modified_base 12: mod_base = OTHER; note = 2'-deoxythymidine
  modified_base 13: mod_base = OTHER; note = 2'-O-methyladenosine
  modified_base 14: mod_base = OTHER; note = 2'-fluoroadenosine
  modified_base 15..18: mod_base = OTHER; note = 2'-O-methylguanosine
  modified_base 19: mod_base = OTHER; note = 2'-O-methylcytidine
  modified_base 20: mod_base = OTHER; note = n is R
  modified_base 21: mod_base = OTHER; note = 2'-O-methylguanosine
  modified_base 22: mod_base = OTHER; note = 2'-O-methyluridine
  modified_base 23: mod_base = OTHER; note = 2'-O-methyluridine
  modified_base 1..2: mod_base = OTHER; note = phosphorothioate linkage
  modified_base 2..3: mod_base = OTHER; note = phosphorothioate linkage
  modified_base 3..4: mod_base = OTHER; note = phosphorothioate linkage
  modified_base 20..21: mod_base = OTHER; note = phosphorothioate linkage
  modified_base 21..22: mod_base = OTHER; note = phosphorothioate linkage
  modified_base 22..23: mod_base = OTHER; note = phosphorothioate linkage
ncgtatnacaataaggggcngtt

SEQ ID NO: 94 - RNA, 24 nt, synthetic construct
  source 1..24: mol_type = other RNA
  modified_base 1: mod_base = OTHER; note = 2'-O-methyluridine
  modified_base 2: mod_base = OTHER; note = 2'-O-methylcytidine
  modified_base 4: mod_base = OTHER; note = 2'-O-methyluridine
  modified_base 5: mod_base = OTHER; note = 2'-fluorocytidine
  modified_base 6: mod_base = OTHER; note = 2'-O-methylguanosine
  modified_base 7: mod_base = OTHER; note = 2'-fluorouridine
  modified_base 8: mod_base = OTHER; note = 2'-O-methyladenosine
  modified_base 9: mod_base = OTHER; note = 2'-fluorouridine
  modified_base 10: mod_base = OTHER; note = n is R
  modified_base 11: mod_base = OTHER; note = 2'-O-methyladenosine
  modified_base 12: mod_base = OTHER; note = 2'-O-methylcytidine
  modified_base 13..14: mod_base = OTHER; note = 2'-O-methyladenosine
  modified_base 15: mod_base = OTHER; note = 2'-fluorouridine
  modified_base 16: mod_base = OTHER; note = 2'-O-methyladenosine
  modified_base 17: mod_base = OTHER; note = 2'-fluoroadenosine
  modified_base 18: mod_base = OTHER; note = 2'-O-methylguanosine
  modified_base 19: mod_base = OTHER; note = 2'-fluoroguanosine
  modified_base 20: mod_base = OTHER; note = 2'-O-methylguanosine
  modified_base 21: mod_base = OTHER; note = 2'-fluoroguanosine
  modified_base 22: mod_base = OTHER; note = 2'-O-methylcytidine
  modified_base 23: mod_base = OTHER; note = 2'-fluorouridine
  modified_base 24: mod_base = OTHER; note = 2'-O-methylguanosine
  modified_base 4..5: mod_base = OTHER; note = phosphorothioate linkage
  modified_base 5..6: mod_base = OTHER; note = phosphorothioate linkage
  modified_base 22..23: mod_base = OTHER; note = phosphorothioate linkage
  modified_base 23..24: mod_base = OTHER; note = phosphorothioate linkage
tcctcgtatnacaataaggggctg

SEQ ID NO: 95 - RNA, 26 nt, synthetic construct
  source 1..26: mol_type = other RNA
  modified_base 1: mod_base = OTHER; note = 2'-O-methyladenosine
  modified_base 2: mod_base = OTHER; note = 2'-O-methyluridine
  modified_base 3: mod_base = OTHER; note = 2'-O-methylcytidine
  modified_base 6: mod_base = OTHER; note = 2'-O-methyluridine
  modified_base 7: mod_base = OTHER; note = 2'-fluorocytidine
  modified_base 8: mod_base = OTHER; note = 2'-O-methylguanosine
  modified_base 9: mod_base = OTHER; note = 2'-fluorouridine
  modified_base 10: mod_base = OTHER; note = 2'-O-methyladenosine
  modified_base 11: mod_base = OTHER; note = 2'-fluorouridine
  modified_base 12: mod_base = OTHER; note = n is R
  modified_base 13: mod_base = OTHER; note = 2'-O-methyladenosine
  modified_base 14: mod_base = OTHER; note = 2'-O-methylcytidine
  modified_base 15..16: mod_base = OTHER; note = 2'-O-methyladenosine
  modified_base 17: mod_base = OTHER; note = 2'-fluorouridine
  modified_base 18: mod_base = OTHER; note = 2'-O-methyladenosine
  modified_base 19: mod_base = OTHER; note = 2'-fluoroadenosine
  modified_base 20: mod_base = OTHER; note = 2'-O-methylguanosine
  modified_base 21: mod_base = OTHER; note = 2'-fluoroguanosine
  modified_base 22: mod_base = OTHER; note = 2'-O-methylguanosine
  modified_base 23: mod_base = OTHER; note = 2'-fluoroguanosine
  modified_base 24: mod_base = OTHER; note = 2'-O-methylcytidine
  modified_base 25: mod_base = OTHER; note = 2'-fluorouridine
  modified_base 26: mod_base = OTHER; note = 2'-O-methylguanosine
  modified_base 1..2: mod_base = OTHER; note = phosphorothioate linkage
  modified_base 6..7: mod_base = OTHER; note = phosphorothioate linkage
  modified_base 7..8: mod_base = OTHER; note = phosphorothioate linkage
  modified_base 24..25: mod_base = OTHER; note = phosphorothioate linkage
  modified_base 25..26: mod_base = OTHER; note = phosphorothioate linkage
atccctcgtatnacaataaggggctg

SEQ ID NO: 96 - RNA, 26 nt, synthetic construct
  source 1..26: mol_type = other RNA
  modified_base 1: mod_base = OTHER; note = 2'-O-methyladenosine
  modified_base 2: mod_base = OTHER; note = 2'-O-methyluridine
  modified_base 3..4: mod_base = OTHER; note = 2'-O-methylcytidine
  modified_base 6: mod_base = OTHER; note = 2'-O-methyluridine
  modified_base 7: mod_base = OTHER; note = 2'-fluorocytidine
  modified_base 8: mod_base = OTHER; note = 2'-O-methylguanosine
  modified_base 9: mod_base = OTHER; note = 2'-fluorouridine
  modified_base 10: mod_base = OTHER; note = 2'-O-methyladenosine
  modified_base 11: mod_base = OTHER; note = 2'-fluorouridine
  modified_base 12: mod_base = OTHER; note = n is R
  modified_base 13: mod_base = OTHER; note = 2'-O-methyladenosine
  modified_base 14: mod_base = OTHER; note = 2'-O-methylcytidine
  modified_base 15..16: mod_base = OTHER; note = 2'-O-methyladenosine
  modified_base 17: mod_base = OTHER; note = 2'-fluorouridine
  modified_base 18: mod_base = OTHER; note = 2'-O-methyladenosine
  modified_base 19: mod_base = OTHER; note = 2'-fluoroadenosine
  modified_base 20: mod_base = OTHER; note = 2'-O-methylguanosine
  modified_base 21: mod_base = OTHER; note = 2'-fluoroguanosine
  modified_base 22: mod_base = OTHER; note = 2'-O-methylguanosine
  modified_base 23: mod_base = OTHER; note = 2'-fluoroguanosine
  modified_base 24: mod_base = OTHER; note = 2'-O-methylcytidine
  modified_base 25: mod_base = OTHER; note = 2'-fluorouridine
  modified_base 26: mod_base = OTHER; note = 2'-O-methylguanosine
  modified_base 1..2: mod_base = OTHER; note = phosphorothioate linkage
  modified_base 6..7: mod_base = OTHER; note = phosphorothioate linkage
  modified_base 7..8: mod_base = OTHER; note = phosphorothioate linkage
  modified_base 24..25: mod_base = OTHER; note = phosphorothioate linkage
  modified_base 25..26: mod_base = OTHER; note = phosphorothioate linkage
atccctcgtatnacaataaggggctg

SEQ ID NO: 97 - RNA, 23 nt, synthetic construct
  source 1..23: mol_type = other RNA
  modified_base 1: mod_base = OTHER; note = n is B33
  modified_base 2: mod_base = OTHER; note = 2'-deoxycytidine
  modified_base 3: mod_base = OTHER; note = 2'-O-methylguanosine
  modified_base 4: mod_base = OTHER; note = 2'-O-methyluridine
  modified_base 5: mod_base = OTHER; note = 2'-deoxyadenosine
  modified_base 6: mod_base = OTHER; note = 2'-O-methyluridine
  modified_base 7: mod_base = OTHER; note = n is 2'-deoxy-R
  modified_base 8: mod_base = OTHER; note = 2'-O-methyladenosine
  modified_base 9: mod_base = OTHER; note = 2'-O-methylcytidine
  modified_base 10..11: mod_base = OTHER; note = 2'-O-methyladenosine
  modified_base 12: mod_base = OTHER; note = 2'-O-methyluridine
  modified_base 13: mod_base = OTHER; note = 2'-O-methyladenosine
  modified_base 14: mod_base = OTHER; note = 2'-fluoroadenosine
  modified_base 15..18: mod_base = OTHER; note = 2'-O-methylguanosine
  modified_base 19: mod_base = OTHER; note = 2'-O-methylcytidine
  modified_base 20: mod_base = OTHER; note = n is R
  modified_base 21: mod_base = OTHER; note = 2'-O-methylguanosine
  modified_base 22: mod_base = OTHER; note = 2'-O-methyluridine
  modified_base 23: mod_base = OTHER; note = 2'-O-methyluridine
  modified_base 1..2: mod_base = OTHER; note = phosphorothioate linkage
  modified_base 2..3: mod_base = OTHER; note = phosphorothioate linkage
  modified_base 3..4: mod_base = OTHER; note = phosphorothioate linkage
  modified_base 20..21: mod_base = OTHER; note = phosphorothioate linkage
  modified_base 21..22: mod_base = OTHER; note = phosphorothioate linkage
  modified_base 22..23: mod_base = OTHER; note = phosphorothioate linkage
ncgtatnacaataaggggcngtt